European Patent Specification EP 3 289 089 B1, published March 1, 2023. Title: CONTROLLING FUNGAL PATHOGENS BY DISABLING THEIR SMALL RNA PATHWAYS USING RNAi-BASED STRATEGY. Applicant: The Regents of the University of California. Application EP 16787063.3. The sequence listing filed with the application follows.

SEQUENCE LISTING (66 sequences)

SEQ ID NO: 1 - DNA, 5529 bp, Botrytis cinerea
atgacgagagacgcagcagcagcaaaaagtctctaccattggcgaagaaaaggcgtcactccttcagccgaagaggatcttctatcgtttgatgatattgttactgccgttccacctacaatcttgtcttcgtctgtcgctccatatacttctcgagataagataccttctgcatctggcaacggagatgctatagcagatgttagcagtggttacctcaaacaggctaccgtatcttctcattctgctcaagtccgatcatcttcaaacggcaatcaaggtgatgccaaaagttctccctctctttcacctgatagtaaactggaattcatctttgggcctcctttaagggagccagagaagccattctttaataaatcttcttattcgtttcgagattcgagagggttgagcagaaatcgggcttcttcttctatggaaaattcgagaactctcgatccaaagatactcaaaccagttatcatcaataatcaccagggcgaatgcttccaagaggcttccagaacaggtatacctcaggctgatacttttgataaatcttcccttgctaagactgcggatatggatttgtcaccagtttctcaccatgcggatgtgcttgcgacgacggtcactgcacagcattctgcaatagccgcccagaacgcagctcaaagctctaagatgccaggtcctgaagcttttttacttgccgaaaaggacgaggcaggttctcccgttgttatatcactgggttctgcaaaccaaattccttctggaaacatttctttgcagcttgattcaccatctctggaaaaccattctccaaatgtgaccccaatcaacaaagtccctacaccattcgcactttctacaaggacaaccgatgacgttttcgcagaacttaggcggcctttgcatccccaagctattcagagccagattgatatcaagacttcctcttgtgttgatagttataacacgaatgatgagattctagacaacaatcaaggttccaatcaaaaagatctgcatgttgttgaaaaggataaggaagaggaagaggaagaggatatgaaccaagccatacccgatatcaaacgtatctcagcacgaaaacaaaagaacgctgccatatttgacgtttttcttaaggaagctaccaaactaccaaagacagaaaagacttcacatgcgaatgatgaagcaattcagtctactaggtggttgattgaccaagcagaaaaacagcatattatagaaagtcccagggactatcaacttgaattgtttgagaaggcaaagaaacagaacattatagctgtacttgatacaggatctggcaagacattcattgcagttctcttacttcggtggatcatagaccaagagcttgaagatagagctattggcaagcctcatcgtgtttcattcttcctgtggaagaaacgactggatacgaatatggtcattgtctgcactgcagaaattttgcgccaatgcctgcaccattcgtttgttacaatggctcaaataaatctgctaattttcgatgaagcccaccatgcaaagaaggatcatccttatgctaggattattaaagatttttatcgcaatgacacggaaaaggatatcgctctgcctaaaatatttgggatgacagcatcaccggtagatgctagagataatgtcaagaaagctgcggaagaacttgaaggtttgctacacagtcaaatatgtactgcagaagatcccagcttgctgcagtactcaatcaaaggtaaacctgagactcttgcctactatgatcccttgggcccgaaattcaatactcctctttatcttcaaatgctcccgcttctaaaagacaatcctatctttcggaagccatttgtatttgggacagaagccagtagaactctaggatcttggtgtgttgaccagatctggactttctgtcttcaagaagaagagtctaagaaactacaagcaaggacggagcaggcgcatcataagaagagagtcccggagccacttgaagtgctagagaaacgcaaggaacaacttgaacaagccaaatccattgtcgaaaatcacactttcgagccaccacactttgcatcaagattattggatgatttcacaacaaaagttcactattcgaataatttatctactaaagtcgttgctctcttgagtattctcaaagatcgtttccaacgacccaccaatgacaagtgtattgtatttgtcaaagaaagatacaccgcacgccttctagcctcacttctctccacacctgaagctgggacaccattcttgaaggctgcaccgctggttggtactacgtctgcttcagccggggaaatgcatatcacatttagatcacaaactcttactatgcacaactttcgcaatggtaaaatcaactgccttatcgcaacatcagttgctgaagaaggtcttgacattcctgactgtaacctcgttgtcagattcgatttgtacaatacagtcattcagtacattcaatctagaggtcgtgctaggcatatcaattcaaggtactaccatatggtagagagccacaacgaggaacagattcgtacaatcaaagaggttttgaagcatgagaaaatgctaaagctttttgcttctgctcttccagaagatcgaaaattgaccggaaacaacttcaatatggattacttcctcagaaaagaacgaggccacagaatttaccctgtcccgaatagtgacgcaaaacttacttacagaatgagcttaacggtcctatctgccttcgttgactcacttcctcgagccccagagtcggttcttcgagtggattatgtcgtcacaactgtcgataagcagtttatctgtgaggccattttgccagaagaagcacccatacgcggagcaattggtcggccagcaacaactaaacaagtggccaaatgctcagcagcctttgaaacttgtgtgattctgcaccagaaaggatacatcaacgactacctactttctacatttaaaagatcagcacacatgatgagaaatgcacttttggctgtggatggaaagaagcaagaagcttatgatatgcagactaaaccaactttatggtcttcgaaagggaaacaaggcatattttatatgactgtcttgtctctcaaatctccagataatcttgacagagcatctcagccattgggcttactgacaagatcacccttgcctgatttgccagaatttgttcttcatttcggagcagggcgaaactctccaacctcgtgcgtacctctcgcttcctcaattacgctcgaaaaaaacaagcttgaccaagttaatatgttcaccctatgtttattccaagatgtgttcagtaaagcatacaaatcagatccggatagtatgccatactttctggttcctatcaactgcctgaatgctattgtcgactggaaatcacaaaacccaatgtcaataatcgattgggagacagttgaatatgtccaagacttcgagaataagcaagctgataagccatgggagcacaagccatggttaggaaagcctgacgattatttcaaagacaaattcataactgatccctttgacgggtctcgaaaattgtggtccgttggaatcacaaaagaatacagaccattggatccagtcccaccaaacacggcgcccaggaagggagctagaaagaacaatagtaatatcatggagtatagttgtagtctctgggcaaaggctagagcaaaacgaacttttgatgaagaacagcctgttattgaagcaacctacatttcacttcggagaaatttgcttgatgaatttgatggaggtgagctcgagacttcaaagaagagttttattattttagaaccattgaaggtatcacctcttccaactaccgtgggtgcaatggcctatcttttacctgcaattattcatcgagttgagtcatatctcattgctcttgaagcaacagacttgttacatcttgatatccgtcctgatcttgcgctagaggctgttaccaaggattccgacaattctggagagcatggtgaggaacagacaaactttcaacgtggaatgggcaataattatgaacgattggaatttcttggggactgcttcttgaagatgggaacgtcaatatctctatacggtctaaatcctgatagtgatgaattccgctaccatgttgatcgtatgtgtctgatttgcaacaaaaatctgttcaatacggctttgaaattagagctttacaaatacattcggtcggcagccttcaaccgacgagcttggtatcccgaaggccccgaattattaagaggaaagacagccacggcaccaaatacccacaagctcggcgataagtcagttgcagatgtttgtgaagcaatgattggagctgctttactaagccaccacgaaagcaagtccatggataatgcggttcgcgccgttactgaagttgtcaatagtgacaaccacaatgctgttgtatggtctgattattacaaattgtatgagaaaccaaaatggcaaactgctacagctacagctgcacaaatagatatggcaagacaagttgaaatgaaacatccatatcatttcaaacacccacgcctgttaagatcagctttcatccatccggcatacttgttcatctatgaacaaattccttgttatcaacgtctcgaatttttgggtgattcgctactcgatatggcatgtgtcaacttcctttttcacaaccacccaacaaaagatcctcagtggctcactgagcacaagatggctatagtatccaatcagtttcttggagctctttgtgtcaaattaggcttccacaaacatctactgacactcgattctcaagttcaaaaaatgattgcagattactcctcagatatcaatgaagctctcattcaagccaaaacggacgcaaagagagtcggcaaagtagaagatgattacgctcgtgattattggattgccgtccgtcaacctcctaaatgtcttcccgatattgtagaagcattcattggtgccatttttgtcgactctgagtatgactacggtgaagttgagaagttctttgaaatgcatatcagatggtactttgaggatatgggcatctacgatacctatgctaacaagcacccaaccactttccttactaatttcttgcaaaagaacatgggatgtgaggactgggcaccagttagtaaggaagtacctggagaggatggtagaaagaatgttgtagtttgcggggtcatcatacacaataaggtggtatcaactgccactgccgaaagtatgagatatgctagggtcggagcagcgaggaatgccttgagaaaattggagggaatgagtgtccgagaattcagggatgaatacgggtgctcatgtgaaggtgatgttgttgatgaagagggcaatattgaatttgttgaacgtgaagacgggatggaggggatcggtatgggatattga

SEQ ID NO: 2 - protein, 1842 aa, Botrytis cinerea
MTRDAAAAKSLYHWRRKGVTPSAEEDLLSFDDIVTAVPPTILSSSVAPYTSRDKIPSASGNGDAIADVSSGYLKQATVSSHSAQVRSSSNGNQGDAKSSPSLSPDSKLEFIFGPPLREPEKPFFNKSSYSFRDSRGLSRNRASSSMENSRTLDPKILKPVIINNHQGECFQEASRTGIPQADTFDKSSLAKTADMDLSPVSHHADVLATTVTAQHSAIAAQNAAQSSKMPGPEAFLLAEKDEAGSPVVISLGSANQIPSGNISLQLDSPSLENHSPNVTPINKVPTPFALSTRTTDDVFAELRRPLHPQAIQSQIDIKTSSCVDSYNTNDEILDNNQGSNQKDLHVVEKDKEEEEEEDMNQAIPDIKRISARKQKNAAIFDVFLKEATKLPKTEKTSHANDEAIQSTRWLIDQAEKQHIIESPRDYQLELFEKAKKQNIIAVLDTGSGKTFIAVLLLRWIIDQELEDRAIGKPHRVSFFLWKKRLDTNMVIVCTAEILRQCLHHSFVTMAQINLLIFDEAHHAKKDHPYARIIKDFYRNDTEKDIALPKIFGMTASPVDARDNVKKAAEELEGLLHSQICTAEDPSLLQYSIKGKPETLAYYDPLGPKFNTPLYLQMLPLLKDNPIFRKPFVFGTEASRTLGSWCVDQIWTFCLQEEESKKLQARTEQAHHKKRVPEPLEVLEKRKEQLEQAKSIVENHTFEPPHFASRLLDDFTTKVHYSNNLSTKVVALLSILKDRFQRPTNDKCIVFVKERYTARLLASLLSTPEAGTPFLKAAPLVGTTSASAGEMHITFRSQTLTMHNFRNGKINCLIATSVAEEGLDIPDCNLVVRFDLYNTVIQYIQSRGRARHINSRYYHMVESHNEEQIRTIKEVLKHEKMLKLFASALPEDRKLTGNNFNMDYFLRKERGHRIYPVPNSDAKLTYRMSLTVLSAFVDSLPRAPESVLRVDYVVTTVDKQFICEAILPEEAPIRGAIGRPATTKQVAKCSAAFETCVILHQKGYINDYLLSTFKRSAHMMRNALLAVDGKKQEAYDMQTKPTLWSSKGKQGIFYMTVLSLKSPDNLDRASQPLGLLTRSPLPDLPEFVLHFGAGRNSPTSCVPLASSITLEKNKLDQVNMFTLCLFQDVFSKAYKSDPDSMPYFLVPINCLNAIVDWKSQNPMSIIDWETVEYVQDFENKQADKPWEHKPWLGKPDDYFKDKFITDPFDGSRKLWSVGITKEYRPLDPVPPNTAPRKGARKNNSNIMEYSCSLWAKARAKRTFDEEQPVIEATYISLRRNLLDEFDGGELETSKKSFIILEPLKVSPLPTTVGAMAYLLPAIIHRVESYLIALEATDLLHLDIRPDLALEAVTKDSDNSGEHGEEQTNFQRGMGNNYERLEFLGDCFLKMGTSISLYGLNPDSDEFRYHVDRMCLICNKNLFNTALKLELYKYIRSAAFNRRAWYPEGPELLRGKTATAPNTHKLGDKSVADVCEAMIGAALLSHHESKSMDNAVRAVTEVVNSDNHNAVVWSDYYKLYEKPKWQTATATAAQIDMARQVEMKHPYHFKHPRLLRSAFIHPAYLFIYEQIPCYQRLEFLGDSLLDMACVNFLFHNHPTKDPQWLTEHKMAIVSNQFLGALCVKLGFHKHLLTLDSQVQKMIADYSSDINEALIQAKTDAKRVGKVEDDYARDYWIAVRQPPKCLPDIVEAFIGAIFVDSEYDYGEVEKFFEMHIRWYFEDMGIYDTYANKHPTTFLTNFLQKNMGCEDWAPVSKEVPGEDGRKNVVVCGVIIHNKVVSTATAESMRYARVGAARNALRKLEGMSVREFRDEYGCSCEGDVVDEEGNIEFVEREDGMEGIGMGY

SEQ ID NO: 3 - DNA, 4197 bp, Botrytis cinerea
atggaatacacttcggaacctgacactgacccggatacacgcggtagccttatcgatggtcgagatgggattgaaggggatcttattgctttgacgtctggggaacgacttaatgagactgtagaggatttatgtagtgactcatcaggattgattgttgagaatgaagatgatgataacagcgcaggggagaagggagagattgtgatagtaacaccaagaacataccaactggaaatgttggaagagagtttgaaaaggaatgtcatcgttgcgatggatacaggaagtggcaagacacatgtggccgttctccgaatactagcggaacttgagcggatgaagcctggcaagataatatggtttcttgcgcctaccgttgcgctctgtgctcagcatcacgaatatctccagctgaatattccctctgttttgatcaaaatgcttattggtgctgatggtgtggatcgatggacagagcagagacagtgggatacggtcttgaaggatgtcaaggtagtcgtatcttcctatcaagttcttctagatgcccttacacacggattcgtacgcatggggcgtctgtccttgatcatttttgatgaagcacataattgtgtaaataaagcgccaggggctaaaattatgaaatctttctatcatccgtataaatcgatattcccacttccccacattctgggcctctcggccagccctgtcatgagatccagtccacaatctttaagtgatatcgaggagactttggatgccatttgctgcacgccaaaaatacatcgagcagatcttcgccttcgagtaaagctaccacttctatctattatctactataccccagagtcaaatatcatcgtgacgaaaactgtggcgagcctgagaaagattgtgcaaagtctcaacattttcgaagacccctacgttttgacactaaaaaggagtgatagcgaaaaaagtcaacgtgagctggcgaaagtactcaagagttttaagacatatagtcaaacccaattaaagtcaatcgacaaaactagcaacgagattattcttgtagagctaggcccatgggctgcagattactatatctcaacagtggtgacgagatacttgaaggcaatgtcggcaaaggacactttcattgttgaagattcaccagctgccgagaagctatatattgccaaggctctcagacaagtcgaaatctctccttcaactctctcagatacaggcaaaatttctaacaaggttgaaaagctactggggataattgcgcaacagaagcctcccttttccgctattatatttgtccaagaaagagccacggtgtctgtgctagcccatctattatcgcatcatccattgacaaaggatcgttttaagattggaaccatggttggcacatccttaaatggcaagcgtacagaccaaataggagagcttgtcgatgttaatcaacaaaaagacactttgtcaagtttcaagcgtggaaaaattgatatccttatagctacaaatgtattggaagagggaattgatgttcctgcctgtaatctagtgatctgctttagtaaaccagcaaacctcaaatctttcgtacaaagacgagggcgagcaagacagcaagattctaagctgattcttcttgatgcttcaggtgataaagcgacaaattggcatgagcttgaaagaaaaatgcgagaggagtacggaaaggaaatgcgagaattgcaacacatctacgaaattgagacagctgatgaacagtcggaagatgatagggtcttgcgaatagaaagcactggggctcaattagaccttgacagtgctttaccacatctctatcatttctgttcagtcttaacaacaaaagattttgttgacctcaggccagacttcgtctactcctccgaactgggatcggaatatgttcgagcaaaggtcatcctgcctggatcggtttctaaacccctgcgagtccatgaaagccgcggatcgtggttgagcgagaggtcggctgcaaaagatgcagcgtttgaggcgtattccgcattatacagggggggcttagtgaatgataacctactgcccctgatggtgcacgacaaagtcatcgatgagttgacttcaaagcccgtggatactcgcgcgtctcttctggaggtgaaggaaagattaaatccatggattgacattgctagagcatggaaagaggcagaacaccatgctggaattgttcgcacatcggtaatgatcttcaatgggatgaagctggaactctgtcttccaattgatccaccggcaatacccccattaaagctttattgggatgctgacaccgagttctttgttgactttacaaacgatatcgagatcggcaccagcgagaatatgttggcacaggcgttgaacgataccaatctactattatcagatcgtggtcgtaaagttcacatccagtcacgtcgaacagttgtgcaatttatcttgcttcaagattcgggctcgctcagttcagattgttttccggttgaccccaacggtaatattaaaagtacaggttttatcagagaagtcggtaaactagaatcgccctacatctttgaaaaatggttgcccaatgcaccagaagacgtcccatatctagctgtggttaaagtaagtcgccgtgcagactttttgcacaaggtacagaacgaaaaaccctcgtcattcactaaacaattctcgtctgttctacctgcctcgacatgtgtacaggatgtaatgcccgcacagttgtctcggttcggcatgatgattccttccatcacacaccacattgaggtgcaactcgttgtagaccgactatccaggaccatcctcaaggatctcgaaattagtgaccagagtcttattcagaccgccatcacacatgccagttattcgttagactcgaattatcagcgtctcgaatttctgggcgactcaattctcaaattgtgtacatcggtacaattggtggcagagcatctagattggcacgaaggatatttgtcggctatgaaggatcgtatcgtgtccaattcacggtcatcaagagcggcggctgaagtcggtttggatgagtatataatgaccaagaaattcacaggtgcaaaatggcgaccaatgtacgtggatgatctggtcgtcacagaacaaaaaacaagagaaatgtcctccaaaattctttccgacgttgtggaagcactcatcggcgcatctctccggcccgtcgagcaaatcctcgcatataccttcaccaaaaaatctctcctcgtcgaagccatgacgcacccctcttacaccagcggcacgcaatccctcgagcgactcgagttcctcggcgattccattctcgacaacatcatcgtcacagccatgtggtcgcactcgacgccgctctcccacttccacatgcatctcctgcgctctgcgctcgtcaacgccgatttcctcgcctttctctgcatggaaatgagcatcgaccaaaacgtcaccaatctgaccgaaggaaaaaaccatcgcatccacgaaacccactcgcgacgccgcgtttccctcgtcagttttctccgtcactcaagcgttcgtctctctatctatcaaaaagaagcgctttctcgccatgcagaattgcgcgatcagatcctcgaggcaatatacaccggtgatacattcccctgggctctattatcccgattggacgcgcggaaatttttctccgatatgattgagagtttgctgggcgcggtatggattgatagcggctcgatggaagtgtgcacgcagctgatcgaaagaatgggcgtcctgagatacatgcgacggattttgaaagatggcgtgcgcatcatgcatccgaaggaggaactgggcatcgtggccgattctgaaaacgtcaggtacgttttgcggcgggagaagatgggtggggatgctaccgaggtaaatgcggacgcggatgaagaggtacgcacggagtaccggtgcacagtatttgtgggcggggaggaaattgtagaggtgaggggtggagcgaggaaagaggagattcaggcaagggctgcggagcaggcggtgcggattttgaaggcgaggggtcatgagaagaggaatgggggtgcgggggaggggaaaaagagaaaatcgctggatgaatag

SEQ ID NO: 4 - protein, 1398 aa, Botrytis cinerea
MEYTSEPDTDPDTRGSLIDGRDGIEGDLIALTSGERLNETVEDLCSDSSGLIVENEDDDNSAGEKGEIVIVTPRTYQLEMLEESLKRNVIVAMDTGSGKTHVAVLRILAELERMKPGKIIWFLAPTVALCAQHHEYLQLNIPSVLIKMLIGADGVDRWTEQRQWDTVLKDVKVVVSSYQVLLDALTHGFVRMGRLSLIIFDEAHNCVNKAPGAKIMKSFYHPYKSIFPLPHILGLSASPVMRSSPQSLSDIEETLDAICCTPKIHRADLRLRVKLPLLSIIYYTPESNIIVTKTVASLRKIVQSLNIFEDPYVLTLKRSDSEKSQRELAKVLKSFKTYSQTQLKSIDKTSNEIILVELGPWAADYYISTVVTRYLKAMSAKDTFIVEDSPAAEKLYIAKALRQVEISPSTLSDTGKISNKVEKLLGIIAQQKPPFSAIIFVQERATVSVLAHLLSHHPLTKDRFKIGTMVGTSLNGKRTDQIGELVDVNQQKDTLSSFKRGKIDILIATNVLEEGIDVPACNLVICFSKPANLKSFVQRRGRARQQDSKLILLDASGDKATNWHELERKMREEYGKEMRELQHIYEIETADEQSEDDRVLRIESTGAQLDLDSALPHLYHFCSVLTTKDFVDLRPDFVYSSELGSEYVRAKVILPGSVSKPLRVHESRGSWLSERSAAKDAAFEAYSALYRGGLVNDNLLPLMVHDKVIDELTSKPVDTRASLLEVKERLNPWIDIARAWKEAEHHAGIVRTSVMIFNGMKLELCLPIDPPAIPPLKLYWDADTEFFVDFTNDIEIGTSENMLAQALNDTNLLLSDRGRKVHIQSRRTVVQFILLQDSGSLSSDCFPVDPNGNIKSTGFIREVGKLESPYIFEKWLPNAPEDVPYLAVVKVSRRADFLHKVQNEKPSSFTKQFSSVLPASTCVQDVMPAQLSRFGMMIPSITHHIEVQLVVDRLSRTILKDLEISDQSLIQTAITHASYSLDSNYQRLEFLGDSILKLCTSVQLVAEHLDWHEGYLSAMKDRIVSNSRSSRAAAEVGLDEYIMTKKFTGAKWRPMYVDDLVVTEQKTREMSSKILSDVVEALIGASLRPVEQILAYTFTKKSLLVEAMTHPSYTSGTQSLERLEFLGDSILDNIIVTAMWSHSTPLSHFHMHLLRSALVNADFLAFLCMEMSIDQNVTNLTEGKNHRIHETHSRRRVSLVSFLRHSSVRLSIYQKEALSRHAELRDQILEAIYTGDTFPWALLSRLDARKFFSDMIESLLGAVWIDSGSMEVCTQLIERMGVLRYMRRILKDGVRIMHPKEELGIVADSENVRYVLRREKMGGDATEVNADADEEVRTEYRCTVFVGGEEIVEVRGGARKEEIQARAAEQAVRILKARGHEKRNGGAGEGKKRKSLDE

SEQ ID NO: 5 - DNA, 4692 bp, Verticillium dahilae
atgacgactgacgagctctctgttggtctggacgccaccggcatctcaatcctcgcagatggaccggaaaacatatcgtccagcacatcaacatctacgactggaaaggaagatggatacctctgtatcaacagattcactcagaataccgccacgacccaggacaaccagagccgagattctgacgacgatgaggatgactgcggcagccacgatgaagctgacgaagattcagacgaaagacagtacagcatgaccccagaaaggcctcataaaattaccgagaagaagcgcgcagatcatgctgcctttcacgactggcttcagagcaactccagcgagattgctcagtcaacccctcagccggctcaaaacctcaaccacacctccacggccctgatggtacgcgagagtgagaatcgtaagatcatcgaaaatcctcgggagtatcagattgagctcttcgagcgggcgaagcgaaagaacatcattgccgtgttacccactggatcaggaaagaccttaatcgcagcccttcttctgcgacacaccctcgaacaagaaaccgcggatcgacgcgcgggcaagcccaagagaatcgcctttttcctcgtggaaaaggttgctcttgccctccaacagcacgcggttctggagtgcaatctggaatttcccattgaccgggtatgcggtgacatggtacggtcggactggatcaaggagtcatggatgaaaagatgggatgacaacatggtcatggtctgcaccgccgccatccttcagcaatgccttgccagatcattcatccgcatggatcagatcaacctgcttgtcttcgatgaagcacatcacgccaagggaaatcatccgtacgcccggatcatcaaggactactacattacggaacctgacaaagaaaggcgccccaagatcttcggcatgactgcctctccggtggatgccctcaccgacgtcaagattgctgccgctcaactcgaaggtttgttgcatagtgagattgcgacaatcgaggaggactctgtatcattcaaacaaatccagaaagaggtcgtcgaacaagactgcaagtaccctgccctcgaaccacccttcaccaccaatcttcataagaagatccaagaacaggtgcgctacaacaagaacttcgcaaaggcgctgagcaattctttagaaatgtcgagctcccttggcagctggtgtgtcgatcgcttctggcagatatttctgaccgaagaaaccctcgcgagattggcagcgcaaactgcacaagacaacatttttgccgatcgcgccgaaaaggagcgcgttgccattgaggaggtccgcaacatcatcaagcaacatcagttcctcccaatcaccaaaaccctgcaagacttgtcgtccaaagtgctgtgcctcctcggccaactggaattgcgcttcagtgcccctaccgatcacaagtgcatcatcttcgtggagaaacgaaacacagccatgattctggctcacctcctctccttgcctggtattggacctctatatctgaaaccggctgcgcttgtcgggaacccatctgacaacagccctcttgccatgtcgtacaaagagcaagtgatgacaataacaaagttcagacgtggtgaatacaactgtcttctcgccacttctgtggccgaggagggcattgacatcgcagactgcaacattgtcattcgattcgatcttttcaactcggtgattcagtacatacaatccaaaggccgcgctcggcacttgaactcggagtatatttgcatggccgagctaggcaacggcaagcatacaagggcgaagatacaagcaaattatgacctctccctcatccgccaattctgcagcacactgccagaagaccgcaagatcgtgggctgggaccccgaggcagctcttcaccatggcgagcgcgaccataagttccacatcgttccatccaccggggccaaactcacctggaccggcagcctcgtggttctgtcaaattttgcctcttctctacaggtgaacgacgaaacactaagtccttcctatatggtctctctcatcggtagcgagtacatctgcgaggtccagcttccgagcaagtctcccattttgagcgtgtcaggcacgctccaaaagaacaaagcagaggccaggtgctccgcagcgtttgagatgtgcatgaagctcatcaaaggtgggttcatcagcagtcaccttcagccgacgtttaccaggaagctcccggccatgcgaaacgcacgcctagccatcagctccaagaagcgtgaacggtacaatatgagggtcaagccagaggtatggtcacggcgtggaccggcatcctctctgttcctcacagtcctgaagcttcgtacacctggtgcattgaacagaccatcacagccactcgccctcctcacacgagaggcactgccagagcttccaggagttccgctatttttcggtaactgtggtcggtccatagcggaggtagtatctgtggcgaaacccatgcacttggatgaagtacgtctagacagcctcagagtattcaccctgcgcattttcaaagatgtcttcagcaaggtatacgattctcaagtcgcagaccttccatacttcctggcacctgctgctcatgaccacagtcatgagttctcaccgaatgaagacccagggtcactgatcgactggagccatctgctgtcgaccaaagaggttgagtacttgccttgggatgaagatcacagtcccagcttctatcaaagcaagtttgtgattgatccatacacgggatcgcgcaagctgtttctcagaggtattcggacagatctcaagccgaccgacttggttccagatggagttcccgaacccacattcaggctctggaaggacgttgagcataccataaaggaatacagcatcagcctctgggcaaagagtcgagcccggagagctggcgaatggttggacactcaacccgtggtagaagccgagttggtctcgctgcgccggaatcttctcgacgaatttgccgattccaagcatgaagggtctagggtctgttatgtgattctccagccgctacagatctcaacactccctgtcgaggtcgtcgctatggcctacaactttcccgccatcatccatcggattgaatcgaatatgatcgcccttgacgcctgccgtatgttgaaccttcgagttcgtcccgacctggctctcgaggcgatgaccaaagattcaagcaacagtgaagagcacgatcaggaaaagattgatttccaggccggcatgggcaataattatgagcgactcgagtttctcggagactgctttctcaaaatggcaaccaccatcgcactttttactcggatccctgacagcaacgagtttgagtgtcacgtcgagcgaatgcttcttatttgcaaccagaatctgttcaatgtcgcattaaagaagaacttgcaagagtacattcgatcaaagcaattcgatcgacgcagttggtacccccagggtctgaagcagaaggcgggcaaagcccaaggagcacaaaactcacactcattggccgacaagtctattgctgatgtatgcgaggccatcattggcgcctcatatttgtcgtacactgacgagggcaactttgacatggccgtacgcgctgtgacggccgtcgtgaggaacaaaaatcacgacatgaaatcatacgaggactattacaaagcatttaagatgccgatctggcaagcggcggagccaagtgctgtgcagatggaagcgtctttacagattaaagagcagatgggatatgagttcaagtctcctgccctgctgcggagtgccttcaagcacccgtcctacccccgtcagtttgagagcgtgcccaattatcagcgcctcgagttcctcggtgacgcgcttctagacatggtctgcgtagactttctcttcaggaagtttcccgacgccgatcctcaatggctcactgaacacaagatggccatggtttcgaaccacttcctcggaagtctgagtgtagagttgggcttctaccggcgtgtccttcactttaacagcatcatggccaatcaaatcaaggactacgtcgacgcacttactcatgcacgccaagaagccgaagcggtggcccagatctctggcacagtctcgcgagattactggctcaacgtgaagcacccccccaaattcctctcagacgtggtcgaggcatacatcggtgctattttcgttgattcaggatacgattatggccaggtacaggcgttcttcgagaagcatatccggcctttcttcgcagacatggcgctatatgattcctttgccagcagccaccctgtcacaacgctggcgcgtatgatgcagcaggactttggctgccaggactggcggcttcttgtaagtgaactgccgccgagctgcgaagacggcggggcagctgcgatcactgagacggaagtgatttgtgggttcatggtccacggaagaatcctgctacatgccaagtcgtcgagtggacggtacgccaaagtgggtgctgcaaagagagcggtcgagaagctcatgggtctcggcaacgacaaagaggtctttcggacggacttcggctgtgactgtgactgtgaaggtcaagcaatctag

SEQ ID NO: 6 - protein, 1563 aa, Verticillium dahilae
MTTDELSVGLDATGISILADGPENISSSTSTSTTGKEDGYLCINRFTQNTATTQDNQSRDSDDDEDDCGSHDEADEDSDERQYSMTPERPHKITEKKRADHAAFHDWLQSNSSEIAQSTPQPAQNLNHTSTALMVRESENRKIIENPREYQIELFERAKRKNIIAVLPTGSGKTLIAALLLRHTLEQETADRRAGKPKRIAFFLVEKVALALQQHAVLECNLEFPIDRVCGDMVRSDWIKESWMKRWDDNMVMVCTAAILQQCLARSFIRMDQINLLVFDEAHHAKGNHPYARIIKDYYITEPDKERRPKIFGMTASPVDALTDVKIAAAQLEGLLHSEIATIEEDSVSFKQIQKEVVEQDCKYPALEPPFTTNLHKKIQEQVRYNKNFAKALSNSLEMSSSLGSWCVDRFWQIFLTEETLARLAAQTAQDNIFADRAEKERVAIEEVRNIIKQHQFLPITKTLQDLSSKVLCLLGQLELRFSAPTDHKCIIFVEKRNTAMILAHLLSLPGIGPLYLKPAALVGNPSDNSPLAMSYKEQVMTITKFRRGEYNCLLATSVAEEGIDIADCNIVIRFDLFNSVIQYIQSKGRARHLNSEYICMAELGNGKHTRAKIQANYDLSLIRQFCSTLPEDRKIVGWDPEAALHHGERDHKFHIVPSTGAKLTWTGSLVVLSNFASSLQVNDETLSPSYMVSLIGSEYICEVQLPSKSPILSVSGTLQKNKAEARCSAAFEMCMKLIKGGFISSHLQPTFTRKLPAMRNARLAISSKKRERYNMRVKPEVWSRRGPASSLFLTVLKLRTPGALNRPSQPLALLTREALPELPGVPLFFGNCGRSIAEVVSVAKPMHLDEVRLDSLRVFTLRIFKDVFSKVYDSQVADLPYFLAPAAHDHSHEFSPNEDPGSLIDWSHLLSTKEVEYLPWDEDHSPSFYQSKFVIDPYTGSRKLFLRGIRTDLKPTDLVPDGVPEPTFRLWKDVEHTIKEYSISLWAKSRARRAGEWLDTQPVVEAELVSLRRNLLDEFADSKHEGSRVCYVILQPLQISTLPVEVVAMAYNFPAIIHRIESNMIALDACRMLNLRVRPDLALEAMTKDSSNSEEHDQEKIDFQAGMGNNYERLEFLGDCFLKMATTIALFTRIPDSNEFECHVERMLLICNQNLFNVALKKNLQEYIRSKQFDRRSWYPQGLKQKAGKAQGAQNSHSLADKSIADVCEAIIGASYLSYTDEGNFDMAVRAVTAVVRNKNHDMKSYEDYYKAFKMPIWQAAEPSAVQMEASLQIKEQMGYEFKSPALLRSAFKHPSYPRQFESVPNYQRLEFLGDALLDMVCVDFLFRKFPDADPQWLTEHKMAMVSNHFLGSLSVELGFYRRVLHFNSIMANQIKDYVDALTHARQEAEAVAQISGTVSRDYWLNVKHPPKFLSDVVEAYIGAIFVDSGYDYGQVQAFFEKHIRPFFADMALYDSFASSHPVTTLARMMQQDFGCQDWRLLVSELPPSCEDGGAAAITETEVICGFMVHGRILLHAKSSSGRYAKVGAAKRAVEKLMGLGNDKEVFRTDFGCDCDCEGQAI

SEQ ID NO: 7 - DNA, 3593 bp, Verticillium dahilae
atcactctacgggtaaaagcgctgagagaatgatcatgatgaatttctatcatccacgcaaacaatcggcactatctgttccccacgtcctgggactgaccgcaagccccataatgcgatctaggctcgaaggccttgaggcactggaacagacactggactcggtttgcgttacgcccagattgcaccgagatgacttaatgacccatgtcaaaaggcccaccgtctgttatgtccattacgaaacgacagatgctaaggatgagcccaagccggtcagcatttcaagtcttcgcgaagcatgcagaaatatggacatcaggcaagatccatacgttatctgtctaagagacaaaggcactgatcgagcacgacgtgagctcatcaaggtccttacaagccataaaacagattcgcaacagcaaatgaagtctttcttcaatcaaagcttgcgagtcctgcgagatctcgggccctgggcggccgagtactacatttggaaggttgttacagattttctggcaatcattgaagcaagagatcaccgcatgaatcaacggaataccgaagaaaagcagtatctggccaacatccttcgacaaatcagtatcagcgagccgccagtcagcatgttgagtgctcataacacgtcgaacaaagtaatggtgctcatggaatacttgtcatctaaagctaccgatggtactgtcgggatcatatttgtcaaagagcgatcaactgcggcgatgcttgcacacgtgattgagtcgcatccactgacacagaataggcactcgagcgttggggttgttgttggtgcttccactcatctggtaaggaagaaagacatgtgggatctgtctcgagcagcccacgagacagagccccttcttcagttcagatctggccacctcaatttgctcatcgccacgagtgtgcttgaagagggcatcgacgttcctgcctgcaacctcgtgatctgttttgatgagcccgagaatctcaaagcctttgtccagcggcgcggccgagcccggaagaaggattctagcctcgtggttcttctccccgggacagaccacgtgcctcaggactgggaaagcatggaagcgacaatgaggacacactacgagagagaacagcgcgaaatacaaatcatggagcagatcgaagcatccgagtctgcaaagtacgaagagtacgttgtcgagagtactaatgccagactcgacttcgagaacgccaaagcgcatctcagcaacttttgtgggcagctctctcccggggagtttatagacaagaggcccgaatacataccccgtgtggtagacaacggagtacctccatctctgagggtcacggtactgttgccaagctatgttccagctgccgtccgccatgctgagagtcgtcgaagctggaagtcggagcatcaggcctcaaaggatgccgcttttcaggcatacgtggctctttacaaagcgggactggtcaatgaacacatgcttccactcacggtaaaagatatcgtacccgcaaacgaacctcgagtagcaaccttgcaggtcaatggcctcttgaatgtctggcttggtattgcccaggcctggatcacgagcactgaaacctggttaactccagtgcacctccgagacgcgacgggattgacgcgaggaacgtatatcatgagaatgccggtagcattgccggcactgccttccacgccggtgtacttcgatcgcgaaggaccatggcttctggattttggcccacaagaacgaaaggagaatcttgaaatgcctgatcatacttcagtgctgcttgcactccactttggccatcactggtctattgctcatggtcagcagcaggttatcagcttcgcttcacaagatggcgaactgaatatcaggcaattaagtgcacggggtttcacaaccgcagatgccgaccgagaggaaatgctgtacctggtacgggacgagtcaggatgcccgtatgtgtacgaccactttctaaatggcaagccgtcacttgaacttgttcaacgacctttccggcgcatcggggactctccaggctttcaagacgcacccagtaacatcccctacttggctctcagaaagtggccgcggtacctggccctcttgcaccaacagaaggtcaacgatctactgccacaggcgacaaacaagaagccatatgctagggtttatccggcaccgtgggcgaaagtcgacacgattccattagatcatgcttactttggggcgttgatccctttcatttcacacattgtcgaggttcgactggttgcagaacagctttcctcgagcctacttcgtgacctcaatttctcagatccctctcttgtcctggcggccattagcactaagggttccttggaagccacaaactacgagcgccttgagcttttgggtgactctatcctcaagctttgcaccacggccaatgccgccgctctgcatggcttagtgtcgaactcgagattgtgtagggctgcactggatgctggccttgacaaatttgttctaactgaaaacttcacttgtcgcacgtggcgccctatctacgtcaacgacatgatggaaaagggtgctcgcgactcaggaccccgtatcatgtcgacgaagacgctcgccgatattgtggaagcactcataggggccgcatacattgacggtggcctcccaaaggcacttgggtgcatttcgatcttcctgagggagctcgattggaaaccgttgccagcttgccaggagatcctttacagtttggcgtcccctgatgtgcctttgccgccaatgcttgttccgctggaggacctgatcggctacacgatgcatctcctcaagactgcttcggtcaacggcgatcttctaggcttccttgcactcgagtgccatgccgaggaagacgaggtgatcattgatatcgatttttctccttccgatacggacttcaatcctcaaaattccgccggggtggaacagaagctcaaacagacacgccggaaaatccccctttggaagtttatgcgccactcctcaatagaggttgtgcagcagcagaccaaagctgccagcgttcatgccgatctccgaggacagatcatgcacgctctggaacatgggtcaagctacccctggtctcttctcgcccgtttacatcccgcaaagttcttctccgacatggtcgaagctgtactgggtgccgtctgggtcgattcgggcgacatgggcgcgtgcattcgtgtggcggaacgactgggcattctgcctgtgctctcccgactggcaaaggaggacgttcatgtgctgcatccgaagcaagagctgggagagatcgctggtccccggacagtcaaatatctcctcactttgcccgaggacgcagccggcctgcaaagtgcaacaagaaaatatgcctgcaaggtcatggtcggggatcgctgtgttgcagaggtggatgacggggtcgctcgagatgaggttgagacaaaggctgcagaggttgcggtacagaccttgaagaatgaacaggctgacgcgaaacaagtagcagaacactaa

SEQ ID NO: 8 - protein, 1187 aa, Verticillium dahilae
MIMMNFYHPRKQSALSVPHVLGLTASPIMRSRLEGLEALEQTLDSVCVTPRLHRDDLMTHVKRPTVCYVHYETTDAKDEPKPVSISSLREACRNMDIRQDPYVICLRDKGTDRARRELIKVLTSHKTDSQQQMKSFFNQSLRVLRDLGPWAAEYYIWKVVTDFLAIIEARDHRMNQRNTEEKQYLANILRQISISEPPVSMLSAHNTSNKVMVLMEYLSSKATDGTVGIIFVKERSTAAMLAHVIESHPLTQNRHSSVGVVVGASTHLVRKKDMWDLSRAAHETEPLLQFRSGHLNLLIATSVLEEGIDVPACNLVICFDEPENLKAFVQRRGRARKKDSSLVVLLPGTDHVPQDWESMEATMRTHYEREQREIQIMEQIEASESAKYEEYVVESTNARLDFENAKAHLSNFCGQLSPGEFIDKRPEYIPRVVDNGVPPSLRVTVLLPSYVPAAVRHAESRRSWKSEHQASKDAAFQAYVALYKAGLVNEHMLPLTVKDIVPANEPRVATLQVNGLLNVWLGIAQAWITSTETWLTPVHLRDATGLTRGTYIMRMPVALPALPSTPVYFDREGPWLLDFGPQERKENLEMPDHTSVLLALHFGHHWSIAHGQQQVISFASQDGELNIRQLSARGFTTADADREEMLYLVRDESGCPYVYDHFLNGKPSLELVQRPFRRIGDSPGFQDAPSNIPYLALRKWPRYLALLHQQKVNDLLPQATNKKPYARVYPAPWAKVDTIPLDHAYFGALIPFISHIVEVRLVAEQLSSSLLRDLNFSDPSLVLAAISTKGSLEATNYERLELLGDSILKLCTTANAAALHGLVSNSRLCRAALDAGLDKFVLTENFTCRTWRPIYVNDMMEKGARDSGPRIMSTKTLADIVEALIGAAYIDGGLPKALGCISIFLRELDWKPLPACQEILYSLASPDVPLPPMLVPLEDLIGYTMHLLKTASVNGDLLGFLALECHAEEDEVIIDIDFSPSDTDFNPQNSAGVEQKLKQTRRKIPLWKFMRHSSIEVVQQQTKAASVHADLRGQIMHALEHGSSYPWSLLARLHPAKFFSDMVEAVLGAVWVDSGDMGACIRVAERLGILPVLSRLAKEDVHVLHPKQELGEIAGPRTVKYLLTLPEDAAGLQSATRKYACKVMVGDRCVAEVDDGVARDEVETKAAEVAVQTLKNEQADAKQVAEH

SEQ ID NO: 9 - DNA, 260 bp, Botrytis cinerea
tgcggaagaacttgaaggtttgctacacagtcaaatatgtactgcagaagatcccagcttgctgcagtactcaatcaaaggtaaacctgagactcttgcctactatgatcccttgggcccgaaattcaatactcctctttatcttcaaatgctcccgcttctaaaagacaatcctatctttcggaagccatttgtatttgggacagaagccagtagaactctaggatcttggtgtgttgaccagatctggactttctgtc

SEQ ID NO: 10 - DNA, 296 bp, Botrytis cinerea
tctttaagtgatatcgaggagactttggatgccatttgctgcacgccaaaaatacatcgagcagatcttcgccttcgagtaaagctaccacttctatctattatctactataccccagagtcaaatatcatcgtgacgaaaactgtggcgagcctgagaaagattgtgcaaagtctcaacattttcgaagacccctacgttttgacactaaaaaggagtgatagcgaaaaaagtcaacgtgagctggcgaaagtactcaagagttttaagacatatagtcaaacccaattaaagtc

SEQ ID NO: 11 - DNA, 293 bp, Verticillium dahilae
ggcaagcccaagagaatcgcctttttcctcgtggaaaaggttgctcttgccctccaacagcacgcggttctggagtgcaatctggaatttcccattgaccgggtatgcggtgacatggtacggtcggactggatcaaggagtcatggatgaaaagatgggatgacaacatggtcatggtctgcaccgccgccatccttcagcaatgccttgccagatcattcatccgcatggatcagatcaacctgcttgtcttcgatgaagcacatcacgccaagggaaatcatccgtacgc

SEQ ID NO: 12 - DNA, 319 bp, Verticillium dahilae
acagacacgccggaaaatccccctttggaagtttatgcgccactcctcaatagaggttgtgcagcagcagaccaaagctgccagcgttcatgccgatctccgaggacagatcatgcacgctctggaacatgggtcaagctacccctggtctcttctcgcccgtttacatcccgcaaagttcttctccgacatggtcgaagctgtactgggtgccgtctgggtcgattcgggcgacatgggcgcgtgcattcgtgtggcggaacgactgggcattctgcctgtgctctcccgactggcaaaggaggacgttcatgtgctg

SEQ ID NO: 13 - DNA, 1021 bp, Botrytis cinerea
ctcctggatcaggcagatgaattagggaactgatttcgaccttccagagttctctttgcgtgatgggtcacttgggtttggttgtcggtatgctgtgggttcggaggagttgtcctttctggtttctttgttggatagtcctttttgggtagcttggtgtgatgcatgcgttctgggtgtgggtctcgtgaggtctttttgtatcaagtatttttaagcttttttcttgttctcttctttttctgtattggtaatgcttcttctttatgatattctcccatcgctgctttcgcattttctaggttgtagggtgcttcccacgtgtcttccgccggttggtagcccttccatcgcaccaggtattgcacacctctgcctctttttctatgtgctaaaatcctttccacctcatgctctatgtgatcgtcaatttcttctggcggcggcgggtcggcggtaccctgtcgttcgtgccatggttcgagtaaagagacgtggaatacattgtggatcttgtaggtgggcggtaatctaagttcgtatgcttgcccgctggtttttatacccgtcacgacaaaggggcctataaatcgatcggagaattttttcttaggtcgcagttgtttaatgttctttgtgcttagcatcaccttgtccccgatgctatatcgctgtggtgaccccttcgtagtgttcttgtttttctgattggttgccgatttccagaattctttcagcttttctctttctttctctaaagcgtcgatgcgctcgcgtgctgccggcgcccttccctctaaatcggcgtcctcgccgatataatggaatgtgggttggaacccatacatagcctggaatgggcttgtattggttgtactgtgccatgtcgcgttatatgtgaattcagcaaggggcaatagcgatgcccagtcgtcttgcctatagttggtgtagcaacttatatagtgaatcaaattttggttttgtcgttcggtttgaccgtcggtctgcgggtggaacg

SEQ ID NO: 14 - DNA, 3927 bp, Botrytis cinerea
atggcatccagagctaccgccacaggtcaatctgccggagacaccaacgacatcgagatgaccgacgccccaaaggagatcactatcaacgaaacccttaagatcgccttaccagacaagtaccaaggtagtcgacaagagctcgatactttcctcttacaacttgagatctactttcgattcaatgaggacaagttcactaccaaggaatccaagagtatatgggccgcatcataccttcgaggtgaagcaaccaaatggatccaaccatatttgcgcgactatttcgagcatgacgataaggatcgtatgcaacccacccgaacaatcttcaatagttttgaaggatttaagacagagattcgtagaatcttcggaaattccaacgagttagaggtagcggaagataagatcttcaacctcaagcagacaggatcagcattgaaatatgctacggaatttcgaagatatgctggaacaaccaagtgggacgaaatcgctatcatgagtcactaccgcaagggactcaaaccagaagtcagactggaattagaaagatctgccgagagtacagatctgaacgatctaattcaggactccatcgaatcagatgatcgtctctacagatatcgacaaagccagagatcatacaaaccccaaggaaatcagaagcaagggcgttaccgcaaaaatgagggtagaccacgttacaatccacagagatacggagaccccatggaactagacgccacgcactacacaaacgggaacgatgactcggaaaagagacgaagacgagaaaacaacttatgctttgaatgtggaaaagcagggcaccgagcagcagactgccgaagcaagaagacaggaggaaaaaggggcaacttcaaacctaagttcggcaaaggccaacttaacgctacctttacaatcccagaaaatccaactaaatccgaaaatactgagactttcaccgttgaggaattccagcaattactaaaggaattaccacgaaatcaagagggcatgaatgcaatagacttatgggagcaagagtattacagaaccccaacaccctctgtgacagaagaaagtcatcaggacgaggcagaagcagaccacgccacgatgagctggacagcttgctatgatgaattctgcggaatccatcgatcagataaagaagcaaccggatggtcccctaagaagagaaagacgaagaaccatcagaataatgtaacatgcgaggatttaactcccaatataacttcgcaagaagttcgcaaagttacccagcagttaaatgctacgggacaggcaggacagatatactgcaaggttcagataaatggacacatacaatcagccatgatagattcaggggctacaggaaattttattgcaccggaagctgagacaatcccaatacgaatgggcataacccaacatacagaggttatacagcttgacgttgtgccattgggccaacaacagatcatcttaggaatgccatggttaaaggcacataatccgaaaatagattgggcacaaggaattgtgacatttgatcagtgcaaaagcggtcacagggacacgctagaggcgttcgcgagacgtaacacgcgccaaggagagttgaacgcgaacaacaccggcgacgtaggacacccagtccagggtcctccattaagagcgaaggccagtacacctcctctacaaatgcagaagccaacgacacggcacgaaatcgcaatcgaggcaaaagaaaagcctacgataccagaacagtacaagaattatgaacatgttttcaaagaaccagggatccatgaggctttaccggaacacaagccatgggatcatgagataatattggaggaaggcaagatgcctgtgcacaccccaatttattcaatgtcagccgatgagttaaagaggctcagagagtacatcgacgacaatttagccaagggatggatcagggaatccgcgtcccaagtggccagtccaactatgtggaaggatcgatatccacttccattagctacggaattaagagatcgattaggcggagctacgatatttaccaagatggacctacgtaatggttaccacttgatcagaatgaaggaaggcgaagaatggaaaaccgcttcaaaacaagatacgggctatacgactactttcatgaggcttatgaacaatgtgttgtcacaatatttggatacttgctgtatatgctacttggacgacatcctagtatattcaaacaacaaggttcaacacattaaggacgttagcaacatcctcgaaagcctatccaaggcagacttgctgtgcaaaccaagcaaatgcgaattccatgtcacagagacagaattcttgggattcaccgtatcaagccaagggctcaagatgagcaaaggcaaggttaaggcagtgctcgaatggaagcagccgaccacaatcaaggaagtacaatcctttctagggttcgtcaacttctacagaagattcatcaagggttattcagggattactacacccttgaccacgttaaccagaaaagatcaaggaagcttcgaatggactgccaaagcacaggagtcattcgatacgctcaaacaagcagtggcagaagagccaatactgttgacttttgacccagagaaagaaatcatagtggagacggactcctcggatttcgctataggagcagttctgagccaaccgggccagaatggaaaataccagccaatcgcattctactcccgaaaactatcaccagccgaattgaattacgagatatatgacaaagaattactggcgatagtcgatgcatttagagaatggcgagtgtatttggaaggatcgaaatacacggtacaggtgtatacagatcataagaacttggtttacttcaccacaacgaagcagttaaacagacgacaggtcagatggtcggagaccatggccaactacaatttcagaatttcatatgtcaaaggatcagaaaacgctagagccgacgctcttagccgaaaaccagaatatcaagaaaacaaaacgtacgagtcatacgctatattcaagaaagacggcgaatcactggtttacaatgcaccacagcttgcagcaacacacctgttggaagacaaccacctcaggaaacagatccaatcacactacgacaaggatgctactgccacacgcatacgcaagacaatagaaccaggattcactatagaaaatgataccatatactttcatggaaaagtatacattccgagtcaaatgaccaaggaatttgtgacggaacaacacgggttgccggcacatggacaccaaggaattgcaaggacatttgcaagaatacgggaaatcagttacttcccacgaatgagaacgatagttgaagaagttgttggaaattgtgacacctgcatacgaaacaagtcatcacgacatgctccgtatggtcagctccagaccccagacatgccttctcagccatggaagtccatcacatgggactttgtggtcaaactaccactctcaaaagatcctactacaggaattgagtacgacgcgatactcaatatagtagacaggctaacgaaatttgcatatatgataccattcaaggaaacatgggatgctgagcaactagcatatgtgttcctaaggatcatagtaagcatacacggagtaccagatgagataatctcggatcgagacaagctctttacctcgaaattctggactaccttattagcacttatgggtatcaagagaaagctatcgacatctttccacccacaaacagatggtcaaacagagaggaccaatcagacaatggaagcatatcttagatgctatcgtataaaatcccgataccacaagaagttaatgccgaatcagcgatag

SEQ ID NO: 15 - DNA, 4857 bp, Botrytis cinerea
atggcatccagagatatcgccacaggtcaatctgccggagacaccaacgacatcgagatgaccgatgccccaaaagagatcactatcaacgaaacacttaagatcgccttaccagacaagtaccaaggtagtcgacaagaactcgatactttcctcttacaacttgagatctacttccgattcaatgaggacaagttcactaccaaggaatccaagagtatatgggccgcatcataccttcgaggtgaagcaaccaaatggatccaaccatatttgcgcgactatttcgagcatgacgataaggatcgcatgcaacccacccgaacaatcttcaatagttttgaaggatttaagacagagattcgtagaatcttcggaaattccaacgagttagaggtagcggaagataagatcttcaacctcaagcagacaggatcagcattgaaatatgctacggaatttcgaagatatgctggaacaaccaagtgggacgaaatcgctatcatgagtcactaccgtaagggactcaaaccagaagtcagactggaattagaaagatctgccgagagtacagatctgaacgatctaattcaggactccatcgaatcagatgatcgtctctacagatatcgacaaagccagagatcatacaaaccccaaggaaatcagaagcaagggcgttaccgcaagaatgagggtagaccacgttacaacccacagagatacggagaccccatggaactagacgctacgcactacacaaacgggaacgatgactcagaaaagagacgaagacgagaaaacaacttatgctttgaatgtggaaaagcagggcaccgagcagcagaatgccgaagcaagaagacaggaggaaaaaggggcaacttcaaacctaagttcggcaagggccaacttaatgccacctttgcaatctcagaaaactcaactaaacccgaaaatactgagactttcaccgttgaggaattccagcaattattagaggaattaccacgaaaccaagagggcatgaatgcaatagacttatgggaacaagagtattacagaactccaacaccctctgtgacagaagaaagtcaccaggacgaggcagaagcggaccacgccacgataagctggacagcttgctatgacgaattctgcggaatccatcgatcagataaagaagcaaccggatggttccctaagaagagaaagacgaagaaccatcagaataatgtaacatgcgaggatttaactcccaatataacttcgcaagaagttcgcaaagttacccagcagttaaatgctacgggacaggcaggacagatatactgcaaggttcagataaatggacacatacaatcagccatgatagattcaggggctacaggaaattttattgcaccagaagcggcaaagtacttggaaataccacttcagaggaaacaatacccctatcgattgcagttagttgacggacagctagcagggtctgacggaaagatttcgcaggagacaatcccagtacgaatgagcataacccaacatacagaggttatacagcttgatgttgtgccattgggccaacaacagatcatcttaggaatgccatggttaaaggcacataatccgaaaatagattgggcacaaggagttgtgacatttgatcagtgcaaaagcggtcacagggacacgatagaggcgtccgcgagacgtaacacgcgccaaggagagttgaacgcgaacaacaccggcgacgtaggacacccagtccagggtcctccattaagagcgaaggccagtacacctcctctacaaatgcagaagccaacgacacggcacgaaatcgcaatcgaggcaaaagaaaggcctacgataccagaacagtacaagaaatatgaacatgttttcaaagaaccagggatccatgaggctttaccggaacacaagccatgggatcatgagataatattggaggaaggcaagatgcctgtgcacaccccaatttattcaatgtcagccgatgagttaaagaggctcagagagtacatcgacgacaatttagccaagggatggatcagggaatccgcgtcccaagtggccagtccaactatgtgggtacccaagaaggatggacccgatagactagttgtagactatagaaagcttaacgcactcactaagaaggatcgatatccacttccattagctacggaattaagagatcgattaggcggagctacgatattcaccaagatggacctacgtaatggttaccacttgatcagaatgaaggaaggcgaagaatggaaaaccgctttcaaaacaagatacgggctatacgagtaccaagttatgccattcgggctaaccaacgcaccagctactttcatgaggcttatgaacaatgtgttgtcacaatatttggatacttgctgtatatgctacttggacgacatcctagtatattcaaacaacaaggttcaacacattaaggacgttagcaacatcctcgaaagcctatccaaggcagacttgctgtgcaaaccaagcaaatgcgaattccatgtcacagagacagaattcttgggattcaccgtatcaagccaagggctcaagatgagcaaagacaaggttaaggcagtgctcgaatggaagcagccgaccacaatcaaggaagtacaatcctttctagggttcgtcaacttctacagaagatttatcaagggttattcagggattactacacccttgaccacgttaaccagaaaagatcaaggaagcttcgaatggactgccaaagcacaggagtcattcgatacgctcaaacaagcagtggcagaagaaccaatactgttgacttttgacccagagaaagaaatcatagtggagacggactcctcggatttcgctataggagcagttctgagccaaccgggccagaatggaaaataccagccaatcgcattctactcccgaaaactatcaccagccgaattgaattacgagatatatgacaaagaattactggcgatagtcgatgcatttagagaatggcgagtgtatttggaaggatcgaaatacacggtacaggtgtatacagatcataagaacttggtttacttcaccacaacgaagcagttaaacagacgacaggtcagatggtcggagaccatggccaactacaatttcagaatttcatatgtcaaaggatcagaaaacgctagagccgacgctcttagccgaaaaccagaatatcaagaaaacaaaacgtacgagtcatacgctatattcaagaaagacggcgaatcactggtttacaatgcaccacagcttgcagcaacacacctgttggaagacaaccacctcaggaaacagatccaatcacactacgacaaggatgctactgccacacgcatacgcaagacaatagaaccaggattcactatagaaaatgataccatatactttcatggaaaagtatacattccgagtcaaatgaccaaggaatttgtgacggaacaacacgggttgccggcacatggacaccaaggaattgcaaggacatttgcaagaatacgggaaatcagttacttcccacgaatgagaacgatagttgaagaagttgttggaaattgtgacacctgcatacgaaacaagtcatcacgacatgctccgtatggtcagctccagaccccagacatgccttctcagccatggaagtccatcacatgggactttgtggtcaaactaccactctcaaaggatcctactacaggaattgagtacgacgcgatactcaatatagtagacaggctaacgaaatttgcatatatgataccattcaaggaaacatgggatgctgagcaactagcatatgtgttcctaaggatcatagtaagcatacacggagtaccagatgagataatctcggatcgagacaagctctttacctcaaaattctggactaccttattagcacttatgggtatcaagagaaagctatcgacatctttccacccacaaacagatggtcaaacagagaggaccaatcagacaatggaagcatatcttagatgctatgtaaattatcgacaagacaattgggtagagctattacccatggcacagttcgcatacaatacatcagaaacggaaaccacgaaaatcacaccagcacgagctaattttgggtttaatccacaagcgtataaaatcccgataccacaagaagttaatgccgaatcagcgatagtacaaatcgaacagctgaaagatctccaagagcaactggctcttgatctaagattcatatcttccagaacagcagcgtactacaatacgaaacgtagtatggaacctacgcttaaagagggggataaagtttatttgctacgacgaaacatcgaaaccaagagaccaagcaataaactcgaccacaggaaactaggaccattcaagattgataaggtaataggaacggttaattatcgattgaaattaccagacacaatgaatatccacccagtattccacatatccttgctcgaaccagcaccaccaggagcgccaaatgcgccatttacagaaattgaaccagtcaacccaaacgccatatacgatgtcgaaacaatactagactgcaaatacgtcagaaacaaggtcaagtatttgatcaaatggttagactacccacattcagaaaacacatgggaactcaaggaagatctcagctgccctgagaagctacgggcattccacctgaagtacccacacctgccaataaagcctcaagatccgcttcggacaactcaggcaaagaaggatcgaagaaatcgaaggaagaagaatcaatag

SEQ ID NO: 16 - DNA, 3909 bp, Botrytis cinerea
atggcatccagagctaccgccacaggtcagtctaccggagataccaacgacatcgagatgaccgatgccccaaaggagatcactatcaacgaaacacttaagatcgccttaccagacaagtaccaaggtagtcgacaagagctcgatactttcctcttacaacttgagatctacttccgattcaatgaggacaagttcactaccaaggaatccaagagcatatgggctgcatcatacctccgaggtgaagcaaccaaatggattcaaccatatttgcgcgactatttcgagcatgacgataaggatcgcatgcaacccacccgaacaatcttcaatagttttgaaggatttaagacagagattcgtagaatcttcggaaattccaacgagttagaggtagcggaagataagatcttcaacctcaagcagacaggatcagcattgaaatatgctacggaatttcgaagatatgctggaacaaccaagtgggacgaaatcgctatcatgagtcactatcgtaagggactcaaaccagaagtcagactggaattagaaagatctgccgagagtacagatctgaacgatctaattcaggactccatcgaatcagatgatcgtctctacagatatcgacaaagccagagatcatacaaaccccaaggaaatcagaagcaagggcgttaccgcaaaaatgagggtagaccacgttacaatccacagagatacggagaccccatggaactagacgccacgcactacacaaacgggaacgatgactcggaaaagagacgaagacgagaaaacaacttatgctttgaatgtggaaaagcagggcaccgagcagcagactgccgaagcaagaagacaggaggaaaaaggggcaacttcaaacctaagttcggcaaaggccaacttaacgctacctttacaatcccagaaaatccaactaaatccgaaaatactgagactttcaccgttgaggaattccagcaattactaaaggaattaccacgaaatcaagagggcatgaatgcaatagacttatgggagcaagagtattacagaaccccaacaccctctgtgacagaagaaagtcatcaggacgaggcagaagcagaccacgccacgatgagctggacagcttgctatgatgaattctgcggaatccatcgatcagataaagaagcaaccggatggttccctaagaagagaaagacgaagaaccatcagaataatgtaacatgcgaggatttaactcccaatataacttcgcaagaagttcgcaaagttacccagcagttaaatgctacgggacaggcaggacagatatactgcaaggttcagataaatggacacatacaatcagccatgatagattcaggggctacaggaaattttattgcaccggaagctgtaaagtacttgggaataccacttcaaacgaaacaacacccctatcgattgcaggacacgctagaggcgtccgcgagacgtaacacgcgccaaggagagttgaacgcgaacaacaccggcgacgtaggacacccagtccagggtcctccattaagagcgaaggccagtacacctcctctacaaatgcagaagccaacgacacggcacgaaatcgcaatcgaggcaaaagaaaggcctacgataccagaacagtacaagaaatatgaacatgttttcaaagaaccagggatccatgaggctttaccagaacacaagccatgggatcatgagataatattggaggaaggcaagatgcctgtgcacaccccaatttattcaatgtcagccgatgagttaaaaaggctcagagaatacatcgacgacaatttagccaagggatggatcagggaatccgcgtcccaagtggccagtccaactatgtgggtacccaagaaggatggacccgatagactagttgtagactatagaaagcttaacgcactcactaagaaggatcgatatccacttccattagctacggaattaagagatcgattaggcggagctacgatatttaccaagatggacctacgtaatggttaccacttgatcagaatgaaggaaggcgaagaatggaagaccgctttcaaaacaagatacgggctatacgagtaccaagttatgccgttcgggctaaccaacgcaccagctactttcatgaggcttatgaacaatgtgttgtcacaatacttggatacttgctgtatatgctacttggacgacatcctagtatattcaaacaacaaggttcaacacattaaggacgttagcaacatcctcgaaagcctatccaaggcagacttgctgtgcaaaccaagcaaatgcgaattccatgtcacagagacagacttcttgggattcaccgtatcaagccaagggctcaagatgagcaaagacaaggttaaggcagtgctcgaatggaaacagccaaccacaatcaaggaggtacaatcctttctagggttcgtcaacttctacagaagatttatcaagggttattcagggattactacacccttgaccacgttaaccagaaaagatcaaggaagcttcgaatggactgccaaagcacaggagtcattcgatacgctcaaacaagcagtggcagaagagccaatactattgacttttgacccagagaaagaaatcatagtggagacggactcctcggatttcgctataggagcagttctgagccaaccgggccagaatggaaaataccagccaatcgcattctattcccgaaaactatcaccagctgagttgaattacgagatatatgacaaagaattgctggcgatagtcgatgcatttagagaatggcgagtatatttggaaggatcgaaatacacagtacaggtgtatacagatcataagaacttggtttacttcaccacaacgaagcagttaaacagacgacaggtcagatggtcggagaccatggccaactacaatttcagaatttcatatgtcaaaggatcagaaaacgctagagccgacgctcttagccgaaaaccagaatatcaagaaaacaaaacgtacgagtcatacgctatattcaagaaagacggcgaatcactggtttacaatgcaccacagcttgcagcaacacacctgttggaagacaactaccttaggaaacagatccaatcacactacgacaaggatgctactgccacacgcatacgtaagacaatagaaccaggattcactatagaaaatgataccatatactttcatggaaaagtatacattccgagtcaaatgaccaaggaatttgtgacggaacaacacggattgccggcacatggacaccaaggaattgcaaggacatttgcaagaatacgggaaatcagttacttcccacgaatgagaacgatagttgaagaagttgttggaaattgtgacacctgcatacgaaacaagtcatcacgacatgctccgtatggtcagctccagaccccagacatgccttctcagccatggaagtccatcacatgggactttgtggtcaaactaccactctccaaggatcctactacaggaattgagtacgacgcgatactcaatatagtagacaggctaacgaaatttgcatatatgataccattcaaggaaacatgggatgctgagcaactagcatatgtgttccttaggatcatagtaagcatacacggagtaccagatgagataatctcggatcgagacaagctctttacctcgaaattctggactaccttattagcacttatgggtatcaagagaaagctatcgacatctttccacccacaaacagatggtcaaacagagaggaccaatcagacaatggaagcatatcttagatgctatcgtataaaatcccgataccacaagaagttaatgccgaatcagcgatag

SEQ ID NO: 17 - DNA, 4857 bp, Botrytis cinerea
atggcatccagagctaccgccacaggtcagcctaccggagataccaacgacatcgagatgaccgatgccccaaaggagatcactatcaacgaaacccttaagatcgccttaccagacaagtaccaaggtagtcgacaagagctcgatactttcctcttacaacttgagatctactttcgattcaatgaggacaagttcactaccaaggaatccaagagtatatgggccgcatcataccttcgaggtgaagcaaccaaatggatccaaccatatttgcgcgactatttcgagcatgacgataaggatcgcatgcaacccacccgaacaatcttcaatagctttgaaggatttaagacagagattcgtagaatcttcggaaattccaacgagctagaggtagcggaagataagatcttcaacctcaagcagacaggatcagcattgaaatatgctacggaatttcgaagatacgctggaacaaccaagtgggacgaaatcgctatcatgagtcactaccgcaagggactcaaaccagaagtcagactggaattagaaagatctgccgagagtacagatctgaacgatctaattcaggactccatcgaatcagatgatcgtctctacagatatcgacaaagccagagatcatacaaaccccaaggaaatcagaagcaagggcgttaccgcaagaatgagggtagaccacgttacaatccacaaagatacggagaccccatggaactagacgctacgcactacacaaacgggaacgatgactcagaaaagagacgaagacgagaaaacaacttatgctttgaatgtggaaaagcagggcaccgagcagcagactgccgaagcaagaagacaggaggaaaaaggggcaacttcaaacctaagttcggcaaaggccaacttaacgctacctttacaatcccagaaaacccaactaaatccgaaaatactgagactttcaccgttgaggaattccagcaattactaaaggaattaccacgaaataaagagggcatgaatgcaatagacttatgggaacaagagtattacagaaccccaacaccctctgtgacagaagaaagtcaccaggacgaggcagaagcggaccacgccacgatgagctggacagcttgctatgatgaattctgcggaatccatcgatcagataaagaagcaaccggatggttccccaagaaaaggaagacgaagaaccatcagaataatgtaacatgcacggatttaacttcaaatataacttcgcgaaaagttcgcaaagttacccagcagttgaatgctacgggacaagcaggacagatatactgcaaggttcagataaatggacacatacaatcagccatgatagattcaggggctacaggaaattttattgcaccagaagctgcaaagtacttggaaataccacttcagacgaaacaatacccctatcgattgcagttagttgacggacagctagcagggtctgacggaaagatttcgcaggagacaatcccagtacgaatgggcataacccaacatacagaggttatacagcttgacgttgtgccattgggccaacaacagatcatcttaggaatgccatggttgaaggcacataatccgaaaatagattgggcacaaggaattgtgacatttgatcagtgcaaaagcggtcacagggacacgctagaggcgtccgcgagacgtaacacgcgccaaggagagttgaacgcgaacaacaccggcgacgtaggacacccagtccagggtcctccattaagagcgaaggccagtacacctcctctacaaatgcagaagccaacgacacggcacgaaatcgcaatcgaggcaaaagaaaggcctacgataccagaacagtacaagaaatatgaacatgttttcaaagaaccagggatccatgaggctttaccggaacacaagccatgggatcatgagataatattggaggaaggcaagatgcctgtgcacaccccaatttattcaatgtcagccgatgagttaaaaaggctcagagaatacatcgacgacaatttagccaagggatggatcagggaatccgcgtcccaagtggccagtccaactatgtgggtacccaagaaggatggacccgatagactagttgtagactatagaaagcttaacgcactcactaagaaggatcgatatccacttccattagctacggaattaagagatcgattaggcggagctacgatattcaccaagatggacctacgtaatggttaccacttgatcagaatgaaggaaggcgaagaatggaaaaccgctttcaaaacaagatacgggctatacgagtaccaagttatgccgttcgggctaaccaacgcaccagctactttcatgaggcttatgaacaatgtgttgtcacaatatttggatacttgctgtatatgctacttggacgacatcctagtatattcaaacaacaaggttcaacacattaaggacgttagcagcatcctcgaaagtctatccaaagcagacttgctgtgcaaaccaagcaaatgcgaattccatgtcacagaaacagaattcttgggattcaccgtatcaagccaagggctcaagatgagcaaagacaaggttaaggcagtgctcgaatggaagcagccgaccacaatcaaggaagtacaatcctttctaggatttgtcaacttctatagaagatttatcaagggttattcagggattactacacccttgaccacgttaaccagaaaagatcaaggaagcttcgaatggactgccaaagcacaggagtcattcgatacactcaaacaagcagtggcagaagaaccaatactgttgacttttgacccagagaaagaaatcatagtggaaacggattcctcagatttcgctataggagcagttctgagccaaccgggccagaatggaaaataccagccaatcgcattctactcccgaaaactatcaccagccgagttgaattacgagatatatgacaaagaattactggcgatagtcgatgcatttagagaatggcgagtatatttggaaggatcgaaatacacagtacaggtgtatacagatcataagaacttggtttacttcaccacaacgaagcagttaaacagacgacaggtcagatggtcggagaccatggccaactacaatttcagaatttcatatgtcaaaggatcagaaaacgctagagccgacgctcttagccgaaaaccagaatatcaagaaaacaaaacgtacgagtcatacgctatattcaagaaagacggcgaatcactggtctacaatgcaccacagcttgcagcaacacacctgttggaagacaaccacctcagaaaacagattcaatcacactacgacaaggatgctactgccacacgcatacgcaagacaatagaaccaggattcactatagaaaatgataccatatactttcatggaaaagtatacattccgagtcaaatgaccaaggaatttgtgacggaacaacatgggttgccggcacatggacaccaaggaattgcaaggacatttgcaagaatacgggaaatcagttacttcccacgaatgagaacgatagttgaagaagttgttggaaattgtgacacctgcatacgaaacaagtcatcacgacatgctccgtatggtcagctccagaccccagacatgccttctcagccatggaagtccatcacatgggactttgtggtcaaactaccactctcaaaggatcctactacaggaattgagtacgacgcgatactcaatatagtagacaggctaacgaaatttgcatatatgataccattcaaggaaacatgggatgctgaacaactagcatatgtgttcctaaggatcatagtaagcatacacggagtaccagatgagataatctcggatcgagacaagctctttacctcaaaattctggactaccttattagcacttatgggtatcaagagaaagctatcgacatctttccacccacaaacagatggtcaaacagagaggaccaatcagacaatggaagcatatcttagatgctatgtaaattatcgacaagacaattgggtagaactattacctatggcacaattcgcatataatacatcggaaacggaaaccacgaaaatcacaccagcacgagctaattttgggtttaatccacaagcgtataaaatcccgataccacaagaagttaatgccgaatcagcaatagtacaagtcgaacagctgaaaaatctccaagagcaactggctcttgatctaagattcatatcttccagaacagcagcgtactacaatacgaaacgtagtatggaacctacgcttaaagagggggataaagtttatttgctacgacgaaacatcgaaaccaagagaccaagcaataaactcgaccacaggaaactaggaccattcaagattgataaggtaataggaacggttaattatcgattgaaattaccagacacaatgaatatccacccagtattccacatatccttgctcgaaccagcaccaccaggagcgccaaatgcgccatttacagaaattgaaccagtcaacccaaacgccatatacgatgtcgaaacaatactagactgcaaatacgtcagaaacaaggtcaagtatttgatcaaatggttagactacccacattcagaaaacacatgggaattcaaggaggatctcagctgccctgagaagctacgggcattccacctgaagtacccacacctgccagtaaagcctcaagatccgcttcggacaactcaggcaaagaaggatcgaagaagtcgaaggaagaagaatcaatag

SEQ ID NO: 18 - DNA, 3909 bp, Botrytis cinerea
atggcatccagagctaccgccacaggtcaatctgccggagacaccaacgacatcgagatgaccgacgccccaaaggagatcactatcaacgaaacccttaagatcgccttaccagacaagtaccaaggtagtcgacaagagctcgatactttcctcttacaacttgagatctactttcgattcaatgaggacaagttcactaccaaggaatccaagagtatatgggccgcatcataccttcgaggtgaagcaaccaaatggatccaaccatatttgcgcgactatttcgagcatgacgataaggatcgtatgcaacccacccgaacaatcttcaatagttttgaaggatttaagacagagattcgtagaatcttcggaaattccaacgagttagaggtagcggaagataagatcttcaacctcaagcagacaggatcagcattgaaatatgctacggaatttcgaagatatgctggaacaaccaagtgggacgaaatcgctatcatgagtcactaccgcaagggactcaaaccagaagtcagactggaattagaaagatctgccgagagtacagatctgaacgatctaattcaggactccatcgaatcagatgatcgtctctacagatatcgacaaagccagagatcatacaaaccccaaggaaatcagaagcaagggcgttaccgcaaaaatgagggtagaccacgttacaatccacagagatacggagaccccatggaactagacgccacgcactacacaaacgggaacgatgactcggaaaagagacgaagacgagaaaacaacttatgctttgaatgtggaaaagcagggcaccgagcagcagactgccgaagcaagaagacaggaggaaaaaggggcaacttcaaacctaagttcggcaaaggccaacttaacgctacctttacaatcccagaaaatccaactaaatccgaaaatactgagactttcaccgttgaggaattccagcaattactaaaggaattaccacgaaatcaagagggcatgaatgcaatagacttatgggagcaagagtattacagaaccccaacaccctctgtgacagaagaaagtcatcaggacgaggcagaagcagaccacgccacgatgagctggacagcttgctatgatgaattctgcggaatccatcgatcagataaagaagcaaccggatggtcccctaagaagagaaagacgaagaaccatcagaataatgtaacatgcgaggatttaactcccaatataacttcgcaagaagttcgcaaagttacccagcagttaaatgctacgggacaggcaggacagatatactgcaaggttcagataaatggacacatacaatcagccatgatagattcaggggctacaggaaattttattgcaccggaagctgtaaagtacttgggaataccacttcaaacgaaacaacacccctatcgattgcaggacacgctagaggcgtccgcgagacgtaacacgcgccaaggagagttgaacgcgaacaacaccggcgacgtaggacacccagtccagggtcctccattaagagcgaaggccagtacacctcctctacaaatgcagaagccaacgacacggcacgaaatcgcaatcgaggcaaaagaaaggcctacgataccagaacagtacaagaaatatgaacatgttttcaaagaaccagggatccatgaggctttaccggaacacaagccatgggatcatgagataatattggaggaaggcaagatgcctgtgcacaccccaatttattcaatgtcagccgatgagttaaaaaggctcagagaatacatcgacgacaatttagccaagggatggatcagggaatccgcgtcccaagtggccagtccaactatgtgggtacccaagaaggatggacccgatagactagttgtagactatagaaagcttaacacactcactaagaaggatcgatatccacttccattagctacggaattaagagatcggttaggcggagctacgatatttaccaagatggacctacgtaatggttaccacttgatcagaatgaaggaaggcgaagaatggaagaccgctttcaaaacaagatacgggctatacgagtaccaagttatgccgttcgggctaaccaacgcaccagctactttcatgaggcttatgaacaatgtgttgtcacaatacttggatacttgctgtatatgctacttggacgacatcctagtatattcaaacaacaaggttcaacacattaaggacgttagcaacatcctcgaaagcctatccaaggcagacttgctgtgcaaaccaagcaaatgcgaattccatgtcacagagacagaattcttgggattcaccgtatcaagccaagggctcaagatgagcaaagacaaggttaaggcagtgctcgaatggaagcagccaaccacaatcaaggaagtacaatcctttctagggttcgtcaacttctacagaagatttatcaagggttattcagggattactacacccttgaccacgttaaccagaaaagatcaagaaagcttcgaatggactgccatagcacaggagtcattcgatacgctcaaacaagcagtggcagaagagccaatactattgacttttgacccagagaaagaaatcatagtggagacggactcctcggatttcgctataggagcagttctgagccaaccgggccagaatggaaaataccagccaatcgcattctactcccgaaaactatcaccagccgaattgaattacgagatatatgacaaagaattgctggcgatagtcgatgcatttagagaatggcgagtatatttggaaggatcgaaatacacagtacaggtgtatacagatcataagaacttggtttacttcaccacaacgaagcagttaaacagacgacaggtcagatggtcggagaccatggccaactacaatttcagaatttcatatgtcaaaggatcagaaaacgctagagccgacgctcttagccgaaaaccagaatatcaagaaaacaaaacgtacgagtcatacgctatattcaagaaagacggcgaatcactggtttacaatgcaccacagcttgcagcaacacacctgttggaagacaactaccttaggaaacagatccaatcacactacgacaaggatgctactgccacacgcatacgcaagacaatagaaccaggattcactatagaaaatgataccatatactttcatggaaaagtatacattccgagtcaaatgaccaaggaatttgtgacggaacaacatgggttgccggcacatggacaccaaggaattgcaaggacatttgcaagaatacgggaaatcagttacttcccacgaatgagaacgatagttgaagaagttgttggaaattgtgacacctgcatacgaaacaagtcatcacggcatgctccgtatggtcagctccagaccccagacatgccttctcagccatggaagtccatcacatgggactttgtggtcaaactaccactctcaaaggatcctactacaggaattgagtacgacgcgatactcaatatagtagacaggctaacgaaatttgcatatatgataccattcaaggaaacatgggatgctgaacaactagcatatgtgttcctaaggatcatagtaagcatacacggagtaccagatgagataatctcggatcgagacaagctctttacctcgaaattctggactaccttattagcacttatgggtatcaagagaaagctatcgacatctttccacccacaaacagatggtcaaacagagaggaccaatcagacaatggaagcatatcttagatgctatcgtataaaatcccgataccacaagaagttaatgccgaatcagcaatag

SEQ ID NO: 19 - DNA, 3909 bp, Botrytis cinerea
atggcatccagagctaccgccacaggtcagtctaccgaagataccaacgacatcgagatgaccgatgccccaaaggagatcactatcaacgaaacacttaagatcgccttaccagacaagtaccaaggtagtcgacaagagctcgatactttcctcttacaacttgagatctacttccgattcaatgaagacaagttcactaccaaggaatccaagagcatatgggctgcatcatacctccgaggtgaagcaaccaaatggattcaaccatatttgcgcgactatttcgagcatgacgataaggatcgcatgcaacccacccgaacaatcttcaatagttttgaaggatttaagacagagattcgtagaatcttcggaaattccaacgagttagaggtagcggaagataagatcttcaacctcaagcagacaggatcagcattgaaatatgctacggaatttcgaagatatgctggaacaaccaagtgggacgaaatcgctatcatgagtcactactgtaagggactcaaaccagaagtcagactagagttagaaagatctgccgagagtacagatctgaacgatctaattcaggactccatcgaatcagatgatcgtctctatagatatcgacaaagccaaagatcatacaaaccccaaggaaaccaaaagcaagggcgttaccgcaagaatgagggtagaccacgttacaatccacagagatacggagaccccatggaactagacgccacgcactacacaaacgggaacgatgactcagaaaagagacgaagacgagaaaacaacttatgctttgaatgtggaaaagcagggcaccgagcagtagactgccgaagcaagaagacaggaggaaaaaggggcaacttcaaacctaagttcggcaagggccaacttaacgccacctttgccatctcagaaaactcaactaaaaccgaaaatactgagactttcaccgttgaggaatttcagcaattactaaaggaattaccacgaaataaagagggcatgaatgcaatagacttatgggaacaagagtattacagaaccccaacaccctctgtgacagaagaaagtcaccaggacgaggcagaagcggaccacgccacgatgagctggacagcttgctatgatgaattctgcggaatccatcgatcagataaagaagcaaccggatggttccccaagaaaaggaagacgaagaaccatcagaataatgtaacatgcgaggatttaactcccaatataacttcgcaagaagttcgcaaagttacccagcagttgaatgctacgggacaggcaggacaagtgtactgcaaggtccagataaatggacacatacaatcagccatgatagattcaggggctacaggaaattttattgcaccagaagctgcaaagtacttggaaataccacttcaaacgaaacaacacccctatcgattgcaggacacgctagaggcgtccgcgagacgtaacacgcgccaaggggagttgaacgcgaacaacaccggcgacgtaggacacccagtccagggtcctccattaagagcgaaggccagtacacctcctctacaaatgcagaagccaacgacacggcacgaaatcgcaatcgaggcaaaagaaaggcctacgataccagaacagtacaagaaatatgaacatgttttcaaagaaccagggatccatgaggctttaccggaacacaagccatgggatcatgagataatattggaggaaggcaagatgcctgtgcacaccccaatttattcaatgtcagccgatgagttaaaaaggctcagagaatacatcgacgacaatttagccaagggatggatcagggaatccgcgtcccaagtggccagtccaactatgtgggtacccaagaaggatggacccgatagactagttgtagactatagaaagcttaacgcactcactaagaaggatcgatatccacttccattagctacggaattaagagatcgattaggcggagctacgatattcaccaagatggacctacgtaatggttaccacttgatcagaatgaaggaaggcgaagaatggaaaaccgctttcaaaacaagatacgggctatacgagtaccaagttatgccattcgggctaaccaacgcaccagctactttcatgaggcttatgaacaatgtgttgtcacaatatttggatacttgctgtatatgctacttggacgacatcctagtatattcaaacaacaaggttcaacacattaaggacgttagcaacatcctcgaaagtctatccaaagcagacttgctgtgcaaaccaagcaaatgcgaattccatgtcacagaaacagaattcttgggattcaccgtatcaagccaagggctcaagatgagcaaagacaaggttaaggcagtgctcgaatggaagcagccaaccacaatcaaggaggtacaatcctttctagggttcgtcaacttctacagaagatttatcaagggttattcagggattactacacccttgaccacgttaaccagaaaagatcaaggaagcttcgaatggactgccaaagcacaggagtcattcgatacactcaaacaagcagtggcagaagaaccaatactgttgacttttgacccagagaaagaaatcatagtggaaacggattcctcagatttcgctataggagcagttctgagccaaccgggccagaatggaaaataccagccaatcgcattctactcccgaaaactatcaccagctgagttaaattacgagatatatgacaaagaattactggcaatagtcgatgcatttagagaatggcgagtatatttggaaggatcgaaatacacagtacaggtgtatacagatcataagaacttggtttacttcaccacaacgaagcagttaaacagacgacaggtcagatggtcggagaccatggccaactacaatttcagaatttcatatgtcaaaggatcagaaaacgctagagccgacgctcttagccgaaaaccagaatatcaagaaaacaaaacgtacgagtcatacgctatattcaagaaagacggcgaatcactggtctacaatgcaccacagcttgcagcaacacacctgttggaagacaaccacctcaggaaacagatccaatcacactacaacaaggatgctactgccacacgcatacgcaagacaatagaaccaggattcactatagaagatgataccatatactttcatggaaaagtatacattccgagtcaaatgaccaaggaatttgtgacggaacaacacggattgccggcacatggacaccaaggaattgcaaggacatttgcaagaatacgggaaatcagttacttcccacgaatgagaacgatagttgaagaagttgttggaaattgtgacacctgcatacgaaacaagtcatcacgacatgctccgtatggtcagctccagaccccagacatgccttctcagccatggaagtccatcacatgggactttgtggtcaaactaccactctcaaaggatcctactacaggaattgagtacgacgcgatactcaatatagtagacaggctaacgaaatttgcatatatgataccattcaaggaaacatgggatgctgagcaactagcatatgtgttcctaagggtcatagtaagcatacacggagtaccagatgagataatctcggatcgagacaagctctttacctcgaaattctggactaccttattagcacttatgggtatcaagagaaagctatcgacatctttccacccacaaacagatggtcaaacagagaggaccaatcagacaatggaagcatatcttagatgctatcgtataaaatcccgataccacaagaagttaatgccgaatcagcaatag

SEQ ID NO: 20 - DNA, 4854 bp, Botrytis cinerea
atggcatccagagctaccgccacaggtcaatctgccggagacaccaacgacatcgagatgaccgacgctccaaaggagatcactatcaacgaaacccttaagatcgccttaccagacaagtaccaaggtagtcgacaagagctcgatactttcctcttacaacttgagatctacttccgattcaatgaggacaagttcactaccaaggaatccaagagcatatgggccgcgtcataccttcgaggtgaagcaaccaaatggattcaaccatatttgcgcgactatttcgagcatgacgataaggatcgcatgcaacccacccgaacaatcttcaatagttttgaaggatttaagacagaggttcgtagaatcttcggaaattccaacgagttagaggtagcggaagataagatcttcaacctcaagcagacaggatcagcattgaaatatgctacggaatttcgaagatatgctggaacaaccaagtgggacgaaatcgctatcatgagtcactaccgcaagggactcaaaccagaagtcagactagaattagaaagatctgccgagagtacagatctaaacgatctaattcaggactccatcgaatcagatgatcgtctctacagatatcgacaaagccaaagatcatacaaaccccaaggaaatcagaagcaagggcgttaccgcaagaatgagggtagaccacgttacaatccacagagatacggagaccccatggaactagacgctacgcactacacaaacgggaacgatgactcagaaaagagacgaagacgagataacaacttatgctttgaatgtggaaaagcagggcaccgagcagcagactgccgaagcaagaagacaggaggaaaaaggggcaacttcaaacctaagttcggcaagggccaacttaatgccacctttgcaatctcagaaaactcaactaaacccgaaaatactgagactttcaccgttgaggaattccagcaattattagaggaattaccacgaaaccaagagggcatgaatgcaatagacttatgggaacaagagtattacagaactccaacaccctctgtgacagaagaaagtcaccaggacgaggcagaagcggaccacgccacgataagctggacagcttgctatgacgaattctgcggaatccatcgatcagataaagaagcaaccggatggttccccaagaagagaaagacgaagaaccgacagaataatgtaacatgcaaggatttaactccaaatgtaacttcgcgaaaagttcgcaaagttacacagcaattgaatgctacgggacaggcaggacaaatatactgcacggttcagataaatggacacatacaatcagccatgatagattcaggggctacagggaattttattgcaccagaagctgcaaagtacttggaaataccacttcaaacgaaacaacacccctaccgattgcagttagttgacggacagctagcagggtctgacggaaagatttcgcaggagacaatcccagtacgaatgggcataacccaacatacagaggttatacagcttgacgttgtgccattgggccaacaacagatcatcttaggaatgccatggttaaaggcacataatccgaaaatagattgggcacaaggaattgtgacatttgatcagtgcaaaagcggtcacagggacacgctagaggcgttcgcgagacgtaacacgcgccaaggagagttgaacgcgaacaacaccggcgacgtaggacacccagtccagggtcctccattaagagcgaaggccagtacacctcctctacaaatgcagaagccaacgacacggcacgaaatcgcaatcgaggcaaaagaaaagcctacgataccagaacagtacaagaattatgaacatgttttcaaagaaccagggatccatgaggctttaccggaacacaagccatgggatcatgagataatattggaggaaggcaagatgcctgtgcacaccccaatttattcaatgtcagccgatgagttaaagaggctcagagagtacatcgacgacaatttagccaagggatggatcagggaatccgcgtcccaagtggccagtccaactatgtgggtacccaagaaggatggacccgatagactagttgtagactatagaaagcttaacgcactcactaagaaggatcgatatccacttccattagctacggaattaagagatcgattaggcggagctacgatatttaccaagatggacctacgtaatggttaccacttgatcagaatgaaggaaggcgaagaatggaaaaccgctttcaaaacaagatacgggctatacgagtaccaagttatgccattcgggctaaccaacgcaccagctactttcatgaggcttatgaacaatgtgttgtcacaatatttggatacttgctgtatatgctacttggacgacatcctagtatattcaaacaacaaggttcaacacattaaggacgttagcaacatcctcgaaagcctatccaaggcagacttgctgtgcaaaccaagcaaatgcgaattccatgtcacagagacagaattcttgggattcaccgtatcaagccaagggctcaagatgagcaaaggcaaggttaaggcagtgctcgaatggaagcagccgaccacaatcaaggaagtacaatcctttctagggttcgtcaacttctacagaagatttatcaaaggttattcagggattactacacccttgaccacgttaaccagaaaagatcaaggaagcttcgaatggactgccaaagcacaggagtcattcgatacgctcaaacaagcagtggcagaagagccaatactattgacttttgacccagagaaagaaatcatagtggagacggactcctcggatttcgctataggagcagttctgagccaaccgggtcagaatggaaaataccagccaatcgcattctactcccgaaaactatcaccagctgagttgaattacgagatatatgacaaagaattactggcgatagtcgatgcatttagagaatggcgagtatatttggaaggatcgaaatacacagtacaggtgtacacagatcataagaacttggtttacttcaccacaacgaagcagttaaacagacgacaggtcagatggtcggagaccatggccaactacaactttagaatttcatatgtcaaaggatcagaaaatgctagagccgacgctcttaaccgaaaaccagaatatcaagaaaacaaagcgtacgagtcatacgctatattcaagaaagacagcgaatcactggtttacaatacaccacagcttgcaacaacacacctgttggaagacaaccacctcaggaaacagatccaatcacactacgacaaggatactactgccacacgcatacgcaaaacaatagaaccaggattcactatagaaaatgataccatatactttcatagaaaagtatacattccgagtcaaatgaccaaggaatttgtgacggaacaacacgggttgccggcacatggacaccaaggaattgcaaggacatttgcaagaatacgggaaatcagttacttcccacgaatgagaacgatagttgaagaagttgttggaaattgtgacacctgcatacgaaacaagtcatcacgacatgctccgtatggtcagctccagaccccagacatgccttctcagccatggaagtccatcacatgggactttgtggtcaaactaccactctcaaaggatcctactacaggaattgagtacgacgcgatactcaatatagtagacaggctaacgaaatttgcatatatgataccattcaaggaaacatgggatgctgagcaactagcatatgtgttcctaaggatcatagtaagcatacacggagtaccagatgagataatctcggatcgagacaagctctttacctcgaaattctggactaccttattagcacttatgggtatcaagagaaagctatcgacatctttccacccacaaacagatggtcaaacagagaggaccaatcagacaatggaagcatatcttagatgctatgtaaattatcgacaagacaattgggtagagctattacccatggcacagttcgcatacaatacatcagaaacggaaaccacgaaaatcacaccagcacgagctaattttgggtttaatccacaagcgtataaaatcccgataccacaagaagttaatgccgaatcagcgatagtacaagtcgaacagttgaaagatctccaagagcaactggctcttgatctaagattcatatcttccagaacagcagcgtactacaatacgaaacgtagtatggaacctacgcttaaagagggggataaagtttatttgctacgacgaaacatcgaaaccaagagaccaagcaataaactcgaccacaggaaactaggaccattcaagattgataaggtaataggaacggttaattatcaattgaaattaccagacacaatgaatatccacccagtattccacatatccttgctcgaaccagcaccaccaggagcgccaaatgcgccatttacagaaattgaaccagtcaacccaaacgccatatacgatgtcgaaacaatactagactgcaaatacgtcagaaacaaggtcaagtatttgatcaaatggttagactacccacattcagaaaacacatgggaactcaaggaagatctcagctgccctgagaaactacgggcattccacctgaagtacccacatctgccaacaaagcctcaagctccgcatcagacaacaaaggcaacgaggggtcgaagaaaccaaaagaagaaccactag

SEQ ID NO: 21 - DNA, 1962 bp, Botrytis cinerea
atgtgggtacccaagaaggatggacccgatagactagttgtagactatagaaagcttaacgcactcactaagaaggatcgatatccacttccattagctacggaattaagagatcgattaggcggagctacgatattcaccaagatggacctactatattcaaacaacaaggttcaacacattaaggacgttagcaacatcctcgaaagcctatccaaggcagacttgctgtgcaaaccaagcaaatgcgaattccatgtcacagagacagaattcttgggattcaccgtatcaagccaagggctcaagatgagcaaaggcaaggttaaggcagtgctcgaatggaagcagccgaccacaatcaaggaagtacaatcctttctagggttcgtcaacttctacagaagatttatcaaaggttattcagggattactacacccttgaccacgttaaccagaaaagatcaaggaagcttcgaatggactgccaaagcacaggagtcattcgatacgctcaaacaagcagtggcagaagagccaatactattgacttttgacccagagaaagaaatcatagtggagacggactcctcggatttcgctataggagcagttctgagccaaccgggtcagaatggaaaataccagccaatcgcattctactcccgaaaactatcaccagctgagttgaattacgagatatatgacaaagaattactggcgatagtcgatgcatttagagaatggcgagtatatttggaaggatcgaaatacacagtacaggtgtacacagatcataagaacttggtttacttcaccacaacgaagcagttaaacagacgacaggtcagatggtcggagaccatggccaactacaactttagaatttcatatgtcaaaggatcagaaaatgctagagccgacgctcttagccgaaaaccagaatatcaagaaaacaaaacgtacgagtcatacgctatattcaagaaagacggcgaatcactggtttacaatgcaccacagcttgcagcaacacacctgttggaagacaaccacctcaggaaacagatccaatcacactacgacaaggatgctactgccacacgcatacgcaagacaatagaaccaggattcactatagaaaatgataccatatactttcatggaaaagtatacattccgagtcaaatgaccaaggaatttgtgacggaacaacacgggttgccggcacatggacaccaaggaattgcaaggacatttgcaagaatacgggaaatcagttacttcccacgaatgagaacgatagttgaagaagttgttggaaattgtgacacctgcatacgaaacaagtcatcacgacatgctccgtatggtcagctccagaccccagacatgccttctcagccatggaagtccatcacatgggactttgtggtcaaactaccactctcaaaggatcctactacaggaattgagtacgacgcgatactcaatatagtagacaggctaacgaaatttgcatatatgataccattcaaggaaacatgggatgctgagcaactagcatatgtgttcctaaggatcatagtaagcatacacggagtaccagatgagataatctcggatcgagacaagctctttacctcgaaattctggactaccttattagcacttatgggtatcaagagaaagctatcgacatctttccacccacaaacagatggtcaaacagagaggaccaatcagacaatggaagcatatcttagatgctatgtaaattatcgacaagacaattgggtagagctattacccatggcacagttcgcatacaatacatcagaaacggaaaccacgaaaatcacaccagcacgagctaattttgggtttaatccacaagcgtataaaatcccgataccacaagaagttaatgccgaatcagcgatatatggaacctacgcttaa

SEQ ID NO: 22 - DNA, 957 bp, Botrytis cinerea
atggccaactacaattttagaatttcatatgtcaaaggatcagaaaacgctagagccgacgctcttagccgaaaaccagaatatcaagaaaacaaaacgtacgagtcatacgctatattcaagaaagacggcgaatcactggtctacaatgcaccacagcttgcagcaacacacctgttggaagacaaccacctcaggaaacagatccaatcacactacaacaaggatgctactgccacacgcatacgcaagacaatagaaccaggattcactatagaagatgataccatatactttcatggaaaagtatacattccgagtcaaatgaccaaggaatttgtgacggaacaacatgggttgccggcacacggacatcaagggattgcaagaacatttgcaagaatccgggaaatcagttacttcccacgaatgagaacgatagttgaagaagttgttggaaattgtgacacctgcatacgaaacaagtcatcacgacatgcgccgtatggtcagctccagaccccagacatgccttctcagccatggaagtccatcacatgggactttgtggtcaaactaccactctcaaaggatcctactacaggaattgagtacgacgcgatactcaatatagtagacaggctaacgaaattcgcatatatgataccattcaaggaaacatgggatgctgagcaactagcatatgtgttcctaaggatcatagtaagcatacacggagtaccagatgagataatctcggatcgagacaagctctttacctcgaaattctggactaccttattagcacttatgggtatcaagagaaagctatcgacatctttccacccacaaacagatggtcaaacagagaggaccaatcagacaatggaagcatatcttagatgctatcgtataaaatcccgataccacaagaagttaatgccgaatcagcgatag

SEQ ID NO: 23 - DNA, 987 bp, Botrytis cinerea
atccaatcacactacaacaaggatgctactgccacacgcatacgcaagacaatagaaccaggattcactatagaagatgataccatatactttcatggaaaagtatacattccgagtcaaatgaccaaggaatttgtgacggaacaacatgggttgccggcacacggacatcaagggattgcaagaacatttgcaagaatccgggaaatcagttacttcccacgaatgagaacgatagttgaagaagttgttggaaattgtgacacctgcatacgaaacaagtcatcacgacatgcgccgtatggtcagctccagaccccagacatgccttctcagccatggaagtccatcacatgggactttgtggtcaaactaccactctcaaaggatcctactacaggaattgacatacacggagtaccagatgagataatctcggatcgagacaagctctttacctcgaaattctggactaccttattagcacttatgggtatcaagagaaagctatcgacatctttccacccacaaacagatggtcaaacagagaggaccaatcagacaatggaagcatatcttagatgctatgtaaattatcgacaagacaattgggtagagctattacccatggcacagttcgcatacaatacatcggaaacggaaaccacgaaaatcaccccagcacgagctaattttgggtttaatccacaagcgtataaaatcccgataccacaagaagttaatgccgaatcagcaatagtacaagtcgaacagctgaaagatctccaagagcaactggctcttgatctaagattcatatcttccagaacagcagcgtactacaatacgaaacgtagtatggaacctacgcttaaagagggggataaagtttatttgctacaacgaaacatcgaaaccaagagaccaagcaataaactcgaccacaggaaactaggaccattcaagattgataaggtaataggaacg

SEQ ID NO: 24 - DNA, 3573 bp, Botrytis cinerea
atggcatccagagccaccgccacaggtcagtctaccggagataccaacgacatcgagatgaccgatgccccaaaggagatcactatcaacgaaacacttaagatcgccttaccagacaagtaccaaggtagtcgacaagagctcgatactttcctcttacaacttgagatctacttccgattcaatgaagacaagttcactaccaaggaatccaagagcatatgggctgcatcatacctccgaggtgaagcaaccaaatggattcaaccatatttgcgcgactatttcgagcatgacgataaggatcgcatgcaacccacccgaacaatcttcaatagttttgaaggatttaagacagagattcgtagaatcttcggaaattccaacgagttagaggtagcggaagataagatcttcaacctcaagcagacaggatcagcattgaaatatgctacggaatttcgaagatatgctggaacaaccaagtgggacgaaatcgctatcatgagtcactaccgtaagggactcaaaccagaagtcagactagagttagaaagatctgccgagagtacagatctgaacgatctaattcaggactccatcgaatcagatgatcgtctctatagatatcgacaaagccaaagatcatacaaaccccaaggaaaccaaaagcaagggcgttaccgcaagaatgagggtagaccacgttacaatccacagagatacggagaccccatggaactagacgccacgcactacacaaacgggaacgatgactcagaaaagagacgaagacgagaaaacaacttatgctttgaatgtggaaaagcagggcaccgagcagtagactgccgaagcaagaagacaggaggaaaaaggggcaacttcaaacctaagttcggcaagggccaacttaacgccacctttgccatctcagaaaactcaactaaaaccgaaaatactgagactttcaccgttgaggaatttcagcaattactaaaggaattaccacgaaataaagagggcatgaatgcaatagacttatgggaacaagagtattacagaaccccaacaccctctgtgacagaagaaagtcaccaggacgaggcagaagcggaccacgccacgatgagctggacagcttgctatgatgaattctgcggaatccatcgatcagataaagaagcaaccggatggttccccaagaaaaggaagacgaagaaccatcagaataatgtaacatgcgaggatttaactcccaatataacttcgcaagaagttcgcaaagttacccagcagttgaatgctacgggacaggcaggacaagtgtactgcaaggtccagataaatggacacatacaatcagccatgatagattcaggggctacaggaaattttattgcaccagaagctgcaaagtacttggaaataccacttcaaacgaaacaacatccctaccgattgcaggacacgctagaggcgtccgcgagacgtaacacgcgccaaggggagttgaacgcgaacaacaccggcgacgtaggacacccagtccagggtcctccattaagagcgaaggccagtacacctcctctacaaatgcagaagccaacgacacggcacgaaatcgcaatcgaggcaaaagaaaggcctacgataccagaacagtacaagaaatatgaacatgttttcaaagaaccagggatccatgaggctttaccggaacacaagccatgggatcatgagataatattggaggaaggcaagatgcctgtgcacaccccaatttattcaatgtcagccgatgagttaaaaaggctcagagaatacatcgacgacaatttagccaagggatggatcagggaatccgcgtcccaagtggccagtccaactatgtgggtacccaagaaggatggacccgatagactagttgtagactatagaaagcttaacgcactcactaagaaggatcgatatccacttccattagctacggaattaagagatcgattaggcggagctacgatattcaccaagatggacctacgtaatggttaccacttgatcagaatgaaggaaggcgaagaatggaaaaccgctttcaaaacaagatacgggctatacgagtaccaagttatgccattcgggctaaccaacgcaccagctactttcatgaggcttatgaacaatgtgttgtcacaatatttggatacttgctatcaaggaagcttcgaatggactgccaaagcacaggagtcattcgatacgctcaagcaagcagtggcagaagaaccaatactgttgacttttgacccagagaaagaaatcatagtggagacggactcctcggatttcgctataggagcagttctgagccaaccgggccagaatggaaaataccagccaatcgcattctactcccgaaaactatcaccagctgagttaaattacgagatatatgacaaagaattactggcaatagtcgatgcatttagagaatggcgagcatatttggaaggatcgaaatacacagtacaggtatatacagatcataagaacttggtttacttcaccacaacgaagcagttaaacagacgacaggtcagatggtcggagaccatggccaactacaactttagaatttcatatgtcaaaggatcagaaaacgctagagccgacgctcttagccgaaaaccagaatatcaagaaaacaaaacgtacgagtcatacgctatattcaagaaagacggcgaatcactggtctacaatgcaccacagcttgcagcaacacacctgttggaagacaaccacctcaggaaacagatccaatcacactacaacaaggatgctactgccacacgcatacgcaagacaatagaaccaggattcactatagaagatgataccatatactttcatggaaaagtatacattccgagtcaaatgaccaaggaatttgtgacggaacaacatgggttgccggcacacggacatcaagggattgcaagaacatttgcaagaatccgggaaatcagttacttcccacgaatgagaacgatagttgaagaagttgttggaaattgtgacacctgcatacgaaacaagtcatcacgacatgcgccgtatggtcagctccagaccccagacatgccttctcagccatggaagtccatcacatgggactttgtggtcaaactaccactctcaaaggatcctactacaggaattgagtacgacgcgatactcaatatagtagacaggctaacgaaatttgcatatatgataccattcaaggaaacatgggatgctgagcaactagcatatgtgttcctaagggtcatagtaagcatacacggagtaccagatgagataatctcggatcgagacaagctctttacctcgaaattctggactaccttattagcacttatgggtatcaagagaaagctatcgacatctttccacccacaaacagatggtcaaacagagaggaccaatcagacaatggaagcatatcttagatgctatcgtataaaatcccgataccacaagaagttaatgccgaatcagcaatag

SEQ ID NO: 25 - DNA, 3909 bp, Botrytis cinerea
atggcatccagagataccgccacaggtcaatctgccggagacaccaacgacatcgagatgaccgatgccccaaaggagatcactatcaacgaaacccttaagatcgccttaccagacaagtaccaaggtagtcgacaagagctcgatactttcctcttacaacttgagatctacttccgattcaatgaggacaagttcactaccaaggaatccaagagtatatgggccgcatcatacctccgaggtgaagcaaccaaatggattcaaccatatttgcgcgactatttcgaacatgacgataagaatcgcatgcaacccacccgaacaatcttcaatagttttgaaggatttaagacagagattcgtagaatcttcggaaattccaacgagttagaggtagcggaagataagatcttcaacctcaagcagacaggatcagcattgaaatatgctacggaatttcgaagatatgctggaacaaccaagtgggacgaaatcgctatcatgagtcactaccgcaagggactcaaaccagaagtcagactggaattagaaagatctgccgagagtacagatctgaacgatctaattcaggactccatcgaatcagatgatcgtctctacagatatcgacaaagccagagatcatacaaaccccaaggaaatcagaagcaagggcgttaccgcaagaatgagggtagaccacgttacaatccacagaggtacggagacccaatggaactagacgctacgcactacacaaacgggaacgatgactcagaaaagagacgaagacgagaaaacaacttatgctttgaatgtggaaaagcagggcaccgagcagcagagtgccgaagcaagaagacaggaggaaaaaggggcaacttcaaacctaagttcggcaagggccaacttaacgccacctttgcaatcccagaaaacccaactaaatccgaaaatactgagactttcaccattgaagaattccagcaattactagaggaattaccacgaaatcaagagggcatgaatgcaatagacttatgggaacaagagtattacagaaccccaacaccctctgtaacagaagaaagtcaccaggacgaggcagaagcagaccacgccacaatgagctggacagcctgctatgatgaattctgcggaattcatcgatcagataaagaagcaaccggatggttccccaagaaaaggaagacgaagaaccatcagaataatgtaacatgcgaggatttaactcccaatacaacttcgcaagaagttcgcaaagttacccagcagttgaatgctacgggacaggcaggacagatatactgcaaagttcagataaatggacacatacaatcagccatgatagattcaggggctacaggaaattttattgcaccagaagctgcaaagtacttggaaataccacttcagacgaaacaacacccctaccgattgcaggacacgctagaggcgtccgcgagacgtaacacgcgccaaggagagttgaacgcgaacgacaccggcgacgtaggacacccagtccagggtcctccattaagagcgaaggccagtacacctcctctacaaatgcagaagccaacgacacggcacgaaatcgcaatcgaggcaaaagaaaagcctacgataccagaacagtacaagaattatgaacatgttttcaaagaaccagggatccatgaggctttaccggaacacaagccatgggatcatgagataatattggaggaaggcaagatgcctgtgcacaccccaatttattcaatgtcagccgatgagttaaaaaggctcagagaatacatcgacgacaatttagccaagggatggatcagggaatccgcgtcccaagtggccagtccaactatgtgggtacccaagaaggatggacccgatagactagttgtagactatagaaagcttaacgcactcactaagaaggatcgatatccacttccattagctacggaattaagagatcgattaggcggagctacgatatttaccaagatggacctacgtaatggttaccacttgatcagaatgaaggaaggcgaagaatggaaaaccgctttcaaaacaagatacgggctatacgagtaccaagttatgccattcgggctaaccaacgcaccagctactttcatgaggcttatgaacaatgtgttgtcacaatatttggatacttgctgtatatgctacttggacgacatcctagtatattcaaacaacaaggttcaacacattaaggacgttagcaacatcctcgaaagcctatccaaggcagacttgctgtgcaaaccaagcaaatgcgaattccatgtcacagagacagaattcttgggattcaccgtatcaagccaagggctcaagatgagcaaaggcaaggttaaggcagtgctcgaatggaagcagccgaccacaatcaaggaagtacaatcctttctagggttcgtcaacttctacagaagatttatcaaaggttattcagggattactacacccttgaccacgttaaccagaaaagatcaaggaagcttcgaatggactgccaaagcacaggagtcattcgatacgctcaaacaagcagtggcagaagagccaatactattgacttttgacccagagaaagaaatcatagtggagacggactcctcggatttcgctataggagcagttctgagccaaccgggtcagaatggaaaataccagccaatcgcattctactcccgaaaactatcaccagccgaattaaattatgaaatatacgacaaagaattactggcaatagtcgatgcatttagagaatggcgagtatatttggaaggatcgaaatacacagtacaggtgtacacagatcataagaacttggtttacttcaccacaacgaagcagttaaacagacgacaggtcagatggtcggagaccatggccaactacaattttagaatttcatatgtcaaaggatcagaaaacgctagagccgacgctcttagccgaaaaccagaatatcaagaaaacaaaacgtacgagtcatacgctatattcaagaaagacggcgaatcactggtttacaatgcaccacagcttgcagcaacacacctgttggaagacaaccacctcaggaaacagatccaatcacactacgacaaggatgctactgccacacgcatacgcaagacaatagaaccaggattcactatagaaaatgataccatatactttcatggaaaagtatacattccgagtcaaatgaccaaggaatttgtgacggaacaacatgggttgccggcacatggacatcaaggaattgcaaggacatttgcaagaatacggggaatcagttacttcccacgaatgagaacgatagttgaagaagttgttggaaattgtgacacctgcatacgaaacaagtcatcacgacatgctccgtatggtcagctccagaccccagacatgccttctcagccatggaagtccatcacatgggactttgtgatcaaactaccactctcaaaggatcctactacaggaattgagtacgacgcgatactcaatatagtagacaggctaacgaaatttgcatatatgataccattcaaggaaacatgggatgctgagcaactagcatatgtgttcctaagggtcatagtaagcatacacggagtaccagatgagataatctcggatcgagacaagctctttacctcgaaattctggactaccttattagcacttatgggtatcaagagaaagctatcgacatctttccacccacaaacagatggtcaaacagagaggaccaatcagacaatggaagcatatcttagatgctatcgtataaaatcccgataccacaagaagttaatgccgaatcagcgatag

SEQ ID NO: 26 - DNA, 288 bp, Botrytis cinerea
atgaccaaggaatttgtgacggaacaacatgggttgccggcacacggacatcaagggattgcaagaacatttgcaagaatccgggaaatcagttacttcccacgaatgagaacgatagttgaagaagttgttggaaattgtacacacctgcatacgaaacaagtcatcacgacatgcgccgtatggtcagctccagaccccagacatgccttctcagccatggaagtccatcacatgggactttgtggtcaaactaccactctcaaaggatcctactacaggaattga

SEQ ID NO: 27 - DNA, 11301 bp, Botrytis cinerea
caaagggggcattacgcttccaactgccgaaaccctgttgtatgtcaacactgtaaaggaagtcacggatccagagagtgcccaggaactatgtcacagccttcccgacagggaaacgcttagacccagctgttattctgagcgtcccactgacgctgggtccccaaatagaaggacgtactacctttaccattatagcaatgttccaaccaaaagataagccgatagcgcttcgatgccttatcgactcaggagcacaagccaacatcatccaacaatccaagtgtatcgaatgggactggctgcctattaagaaaggaacagctttagtatctgcgaacggtaccacgatgccgtcgtatggtaaccatcagttccccgtcgaagtaaaagatcaaaagggagagaagagaaccttcacccacgagtttactgctgctgtactagacttacccaaaatcgatgctatatttggattaccctggctacaagcggtaaacccagatatcgactggaaatcgacgtctcttcactatcgcccctctcttagcgacctcgaaatgatttctgcaagcgaactctatagcgaagtgaaaaagggcgtccatgtatatgttatactaccagagatccagccccattaccgtagagacaacgggtaccgccgggtactcacgctctccacactaaatatccccgaagaataccaagaataccaacaagccttttccgaggaagaaagcagtactctaccagaacaccactcgatggagcatcgcattgatctcgaagccgattcgaaacctccttgggggccaatctattctttatctgaagaggaatcaatagtattaagggaatacttagtagaatatcaaaaaaagggatggataaggaggtccattagttcggcaggagcgccaatcatgtttgttcccaagaaggggggaggctatcggctttgtgtcgactaccggggtctaaataggataaccaaaaaggatcgaaccccgctacccctaatcagcgagtccttagaccgacttcgacaaggtgtcgtcttcactaaattggacctgcgagatgcctaccaccgtattcgtatcagggaaggcgacgaatggaagacggcgttccgcacgcggtacgggcaattcgaatacttagttatgccattcggcctgaccaatgctccagcaacgttccaaacatacatcaatcaagcactgtcaggcttgacagacaccatatgcgtagtgtacctagatgatatcctgatttactctgaggatagagaaagccacacgcgggatgtccgcagggtcctcgaacgccttatagaatacaagctgttcgcaaaactgaaaaaatgtgtcttttacacccatgaggttgaattcctaggattcgtcgtctcgggagcgggagtgacgatggaatccagccgcattcaaactattatagaatggccaacacctacaaaccttagggagctacaggtgttcctgggcttcgcgaacttctatcgacggtttatcaggacctattcgacggtagcccacgggatgaccgcccttatgaagggaacaaagaaaggtaaaatggtaggggagtttatatggacaaaggaggcccaagatgcatttgaggcactaaagaaagcattcaccacggcaccgatactcaagcacttcgaaccatcgctccgcatcatggtcgaaaccgactcgtcggtgtttgctctaggatgcatcctatcgcaactattcgaaggagggactgcagaagcaccgatacgacggtggcaccccgtcgcgttctattcgagaaagctgaaccctgcagaacaacgatacttcactcacgatcaggaattattagcaatatacactgcattcatgcaatggcgccattacttgataggtagtcggcacacaatcgtggtgaaatcggaccataacagcttacaacattttatggtgaaaaagaccctcaatggcagacaagctagatgggcggaagtactagcagcctacgacttcgaaatagtgtacagggcagggaaactgaatccagccgacgggccatcgcgccgccccgactacgctaccgacacggagggtatcaatgatatgctacccacactccagaataaattaaaaagtaccgcagttatcgcgagtttattttacgaatccaccgtgaaaacggaacccctgcgtattgctattagtcgcttgcaaagggaagggtatagcttgccattacgtggacagttagtttcactggtaaaaactggttgcaaacagtcgataccacgtcggattgccagtgttttcgcatccgacgaaacggcattcgaacctatatcggagtcgatgggaaaagctttattgcggcttcagaaagaagacgattttataaagaataaagagtacctaagacaaagattacgttccgccggagacgcctcaccacggcaggtgggcgccgacgagctccttagacacaaggggagcgcgtacgtaccgccagacagcgctctcagagcagaaatcttagaaacgcatcacgatgaccctattggaggtcattggggtgtcgctaaaacattggaaatactgaagtctaaatattattggccttcaatgagaaaagacgtcaaacaacatgtcaaaacatgtgcggtatgccagcgaaccgctatcaaaagacataagccacacggcgagttacagaccctccctattccaaaaggaccctggaaagagataactatggattttattacagatttacctccttcgaaacacggaaaacacgtatacgattctattctagtagtagtcgacaggttcacgaagctagcccgatatatcgccgtcaacaagacgatatcgtctcctgaattagctgacactatggtcagcacagtatttaaagactttggtgtgccagagggcatagtctccgataggggaccgcaattcgtcagtaaattttggagtagcctaatgttttacttgcgaatccgtcgtaagctgtcgacggcgttccacccgcagaccgacggtcaaaccgaacgacaaaaccaaaatttgattcactatataagttgctacaccaactataggcaagacgactgggcatcgctattgccccttgctgaattcacatataacgcgacatggcacagtacaaccaatacaagcccattccaggctatgtatgggttccaacccacattccattatatcggcgaggacgccgatttagagggaagggcgccggcagcacgcgagcgcatcgacgctttagagaaagaaagagaaaagctgaaagaattctggaaatcggcaaccaatcagaaaaacaagaacactacgaaggggtcaccacagcgatatagcatcggggacaaggtgatgctaagcacaaagaacattaaacaactgcgacctaagaaaaaattctccgatcgatttataggcccctttgtcgtgacgggtataaaaaccagcgggcaagcatacgaacttagattaccgcccacctacaagatccacaatgtattccacgtctctttactcgaaccatggcacgaacgacagggtaccgccgacccgccgccgccagaagaaattgacgatcacatagagcatgaggtggaaaggattttagcacatagaaaaagaggcagaggtgtgcaatacctggtgcgatggaagggctaccaaccggcggaagacacgtgggaagcaccctacaacctagaaaatgcgaaagcagcgatgggagaatatcataaagaagaagcattaccaatacagaaaaagaagagaacaagaaaaaagcttaaaaatacttgatacaaaaagacctcacgagacccacacccagaacgcatgcatcacaccaagctacccaaaaaggactatccaacaaagaaaccagaaaggacaactcctccgaacccacagcataccgacaaccaaacccaagtgacccatcacgcaaagagaactctggaaggtcgaaatcagttccctaattcatctgcctgatccaggaggtcagctgcaatatctcgatcgccaagaaggacagaacctacatcgctggcatatcccccgggactcgcgagcccgatctgatcaacctcaccccccccactgatctcatcttgatcaccgactccttcctcctcgttctcgcgaatctcgctgacagggcgagctcctgtcggaaaaccagcggcaacccgttgcctcttggagacccgctccacatcagaattctcagagcgaagcctttggggcgaatctgcttgactatcagactcaccaatatagacttgttgaacagtgctgggagccctctttcgggatttaagagagcctacgggatgagagcggggtgtcggtgtgttgcgagaggcaagctgcgacgacttagaagcggaaaggggaatggcggatctagtcgcgagcttatcggaccgagaacgacgaggcgtagcaggaggagcgttctttctacccaagcttccaaacaataaagccggtacactctcatccaaggggtgacgcggggcaccggtggtctgatgaggttgatccgacacatcatcctcttcaggagcagactcttcggattcattgggatccacgattacactcctcttcaacttcgcagaacctttccggaggccttgctgagccgtcgtgaagacagcggggcccgtccggctcgatgaagcagaagcatgacggcgacctagggaaccagctaccatattcaggccctggttaccacctgggggccccggaggagcttgaacaccctgcagtgcgtcggcgacagcgcgcacagcgcgagggtgtataaccggagccatgaactccccttcttcgtccgagtttaaggcggcgattaatggtgcagtaggagctgcggcggcgacgtccaaggcaggcaggttattctaagaaccatcaaatcagctatcaacagcaccaaggggcaagagcagggcaaccgacaacgaatcgatacgaatccacaatgcgctccataagatcgccaattctactcaatttggacaccagaagaagagtcaattcctctgcggactgcggtttgtgagtccccccttgtttaacctcttttcgaaggaaagcctccactgccttgacgtatcgattacaccggcgaatcaccacctcggaggcgtcctcatcctcttggctattatccggagtaaggcaccaaaaggcatgagtctgatataagaggttcacgtcgggaacaaagcgaggaggtatcgggaggcagactttcttttgtttgcgacaataactacatttagcagcaggacctttatcaaaatggcaaaattcgtcgttagaagagacggcaattcgcttagaacatcgaaggcaagtagggataactaacgcggaaggggccgctgcggaccgatcagcgatagcagccggagcgatgggttgcagtgcagccatcttcgtatgagtaaataagggggaataatctgattgtgggagatatatcagaggcaagaagaccccccttatagaactatcggtgatctgccggtaaggcggtgaggcgcgtaagaatgccgccgtttgcttgtttattgtttgtaatgcctaaacaagattggaattgcttttggaatgcggcgcagggtcgggcatgcagcgacgcgacgacgcgacccacattccgagtaaacaatacggaaggaagcaaacacttctcgggacgcgaagtgtaaagagaggggctctgttacgggacaaaacgtgaccggctcaattaggcacgtgacagtggacctctcgggtctactgcgtgccgaatggggcccgcacacgtataaattgtataatttgcatagttatagaaaagcaatgaaaagtcttggtgccacaatatactagttgattcatttgttacggaggtacccgcaccgcaacatggattataagataaacctaaggccttggtgttggaacctacgaaaacagcactgtagggacagttgaattaaagggtaactaaagatagcagtaaccgaatcaataagcaatgattaaaagataggtacctatcttttgttggcacctaccctacagtaggcacaggagggatagcggttataggttatctagtaagcacaggttagataagcagtagtatcatgtaggtcacggggcaagtgtcacgtgatggatagacaggataggcaggctatccaggctatccgtggatagacaggatagacagtctacccaagctatccagacgagaacgaaggtctatataagggaatgggtttcattacaatgtagagcttcgtgctcaagaacaatcattagtttcattactatagttacgagaattgcaaccagttacaaccttattgaattcctacttgaagtctagtctaaaccacctcgagagatctctagacacttccacgtgaccctagaggcagctcccgtaacactttgagcaccctttctgcttcaagtaccgattcgataaccaaccgctaatatggcatccagagctaccgccacaggtcagtctaccgaagataccaacgacatcgagatgaccgatgccccaaaggagatcactatcaacgaaacacttaagatcgccttaccagacaagtaccaaggtagtcgacaagagctcgatactttcctcttacaacttgagatctacttccgattcaatgaagacaagttcactaccaaggaatccaagagcatatgggctgcatcatacctccgaggtgaagcaaccaaatggattcaaccatatttgcgcgactatttcgagcatgacgataaggatcgcatgcaacccacccgaacaatcttcaatagttttgaaggatttaagacagagattcgtagaatcttcggaaattccaacgagttagaggtagcggaagataagatcttcaacctcaagcagacaggatcagcattgaaatatgctacggaatttcgaagatatgctggaacaaccaagtgggacgaaatcgctatcatgagtcactactgtaagggactcaaaccagaagtcagactagagttagaaagatctgccgagagtacagatctgaacgatctaattcaggactccatcgaatcagatgatcgtctctatagatatcgacaaagccaaagatcatacaaaccccaaggaaaccaaaagcaagggcgttaccgcaagaatgagggtagaccacgttacaatccacagagatacggagaccccatggaactagacgccacgcactacacaaacgggaacgatgactcagaaaagagacgaagacgagaaaacaacttatgctttgaatgtggaaaagcagggcaccgagcagtagactgccgaagcaagaagacaggaggaaaaaggggcaacttcaaacctaagttcggcaagggccaacttaacgccacctttgccatctcagaaaactcaactaaaaccgaaaatactgagactttcaccgttgaggaatttcagcaattactaaaggaattaccacgaaataaagagggcatgaatgcaatagacttatgggaacaagagtattacagaaccccaacaccctctgtgacagaagaaagtcaccaggacgaggcagaagcggaccacgccacgatgagctggacagcttgctatgatgaattctgcggaatccatcgatcagataaagaagcaaccggatggttccccaagaaaaggaagacgaagaaccatcagaataatgtaacatgcgaggatttaactcccaatataacttcgcaagaagttcgcaaagttacccagcagttgaatgctacgggacaggcaggacaagtgtactgcaaggtccagataaatggacacatacaatcagccatgatagattcaggggctacaggaaattttattgcaccagaagctgcaaagtacttggaaataccacttcaaacgaaacaacacccctatcgattgcagttagttgatggacagctagcagggtctgacggaaagatttcgcaggagacaatcccagtacgaatgggcataacccaacatacagaggttatacagcttgacgttgtgccattgggccaacaacagatcatcttaggaatgccatggttgaaggcacataatccgaaaatagattgggcacaaggaattgtgacatttgatcagtgcaaaagcggtcacagggacacgctagaggcgtccgcgagacgtaacacgcgccaaggggagttgaacgcgaacaacaccggcgacgtaggacacccagtccagggtcctccattaagagcgaaggccagtacacctcctctacaaatgcagaagccaacgacacggcacgaaatcgcaatcgaggcaaaagaaaggcctacgataccagaacagtacaagaaatatgaacatgttttcaaagaaccagggatccatgaggctttaccggaacacaagccatgggatcatgagataatattggaggaaggcaagatgcctgtgcacaccccaatttattcaatgtcagccgatgagttaaaaaggctcagagaatacatcgacgacaatttagccaagggatggatcagggaatccgcgtcccaagtggccagtccaactatgtgggtacccaagaaggatggacccgatagactagttgtagactatagaaagcttaacgcactcactaagaaggatcgatatccacttccattagctacggaattaagagatcgattaggcggagctacgatattcaccaagatggacctacgtaatggttaccacttgatcagaatgaaggaaggcgaagaatggaaaaccgctttcaaaacaagatacgggctatacgagtaccaagttatgccattcgggctaaccaacgcaccagctactttcatgaggcttatgaacaatgtgttgtcacaatatttggatacttgctgtatatgctacttggacgacatcctagtatattcaaacaacaaggttcaacacattaaggacgttagcaacatcctcgaaagtctatccaaagcagacttgctgtgcaaaccaagcaaatgcgaattccatgtcacagaaacagaattcttgggattcaccgtatcaagccaagggctcaagatgagcaaagacaaggttaaggcagtgctcgaatggaagcagccaaccacaatcaaggaggtacaatcctttctagggttcgtcaacttctacagaagatttatcaagggttattcagggattactacacccttgaccacgttaaccagaaaagatcaaggaagcttcgaatggactgccaaagcacaggagtcattcgatacactcaaacaagcagtggcagaagaaccaatactgttgacttttgacccagagaaagaaatcatagtggaaacggattcctcagatttcgctataggagcagttctgagccaaccgggccagaatggaaaataccagccaatcgcattctactcccgaaaactatcaccagctgagttaaattacgagatatatgacaaagaattactggcaatagtcgatgcatttagagaatggcgagtatatttggaaggatcgaaatacacagtacaggtgtatacagatcataagaacttggtttacttcaccacaacgaagcagttaaacagacgacaggtcagatggtcggagaccatggccaactacaatttcagaatttcatatgtcaaaggatcagaaaacgctagagccgacgctcttagccgaaaaccagaatatcaagaaaacaaaacgtacgagtcatacgctatattcaagaaagacggcgaatcactggtctacaatgcaccacagcttgcagcaacacacctgttggaagacaaccacctcaggaaacagatccaatcacactacaacaaggatgctactgccacacgcatacgcaagacaatagaaccaggattcactatagaagatgataccatatactttcatggaaaagtatacattccgagtcaaatgaccaaggaatttgtgacggaacaacacggattgccggcacatggacaccaaggaattgcaaggacatttgcaagaatacgggaaatcagttacttcccacgaatgagaacgatagttgaagaagttgttggaaattgtgacacctgcatacgaaacaagtcatcacgacatgctccgtatggtcagctccagaccccagacatgccttctcagccatggaagtccatcacatgggactttgtggtcaaactaccactctcaaaggatcctactacaggaattgagtacgacgcgatactcaatatagtagacaggctaacgaaatttgcatatatgataccattcaaggaaacatgggatgctgagcaactagcatatgtgttcctaagggtcatagtaagcatacacggagtaccagatgagataatctcggatcgagacaagctctttacctcgaaattctggactaccttattagcacttatgggtatcaagagaaagctatcgacatctttccacccacaaacagatggtcaaacagagaggaccaatcagacaatggaagcatatcttagatgctatgtaaattatcgacaagacaattgggtagagctattacccatggcacagttcgcatacaatacatcggaaacggaaaccacgaaaatcaccccagcacgagctaattttgggtttaatccacaagcgtataaaatcccgataccacaagaagttaatgccgaatcagcaatagtacaagtcgaacagctgaaagatctccaagagcaactggctcttgatctaagattcatatcttccagaacagcagcgtactacaatacgaaacgtagtatggaacctacgcttaaagagggggataaagtttatttgctacaacgaaacatcgaaaccaagagaccaagcaataaactcgaccacaggaaaataggaccattcaagattgataaggtaataggaacggttaattatcgattgaaattaccagacacaatgaatatccacccagtattccacatatccttgctcgaaccagcaccaccaggagcgccaaatgcgccatttacagaaatcgaaccagtcaacccaaacgccatatacgacgttgaaacaatactagattgtaaatatgtcaggggcaaaatcaagtatttgatcaaatggttagactacccacattcggaaaacacatgggaa

SEQ ID NO: 28 - DNA, 936 bp, Botrytis cinerea
gaagaggttgttggcaatattttgaagaaagctgaggctgatttgaatggagattaaaaggggaatgaagctgcggggccaccgatagcacaaaaactactgaagatttgaagcacgttaaaattacactcaggaataaacggatggcaagcttttcgatcgcccaaacacggatctacgactacgagttacgcacgacatgatttagccttttgtgtgcaatgatgattagatagcattgcatttctcgaaattgacggcacgacttttacgggcagataatatcaaagattcctagtgagcaagcggtgatgatacgatgtcattccaaaagttttttcctcgcgaattttatttcatttcgaaggcatctttgcttagcagcatattcacctttgatgtcctctgtaggggatggagtctctaatctcgcggtcacaatgagacgtgatgcgctgcgaagtggtgacaatttccctttacttagaatagatcatgcacacatgcatgatgcatagctagctagttttttattcaatgatagtttaatgacaaacacgtatctagatatcctcattcatgtatctgtgggaggttgacttaagttatggctgacttgatagtttcattatatatgtatatgtgatatctaagtaaagattaaagtgaaatcgaaatgcaacgccgaaattctattaattccatgaaatgatgtgatatggcatgacatgatatccaaactccgatttgaaatgctccagcttcgctttctaaaattggtaaaagggacattatttcgtctggttgtgggttttcatttctgtgctcctactaggtgtgaatgatagagtatgctgtggtgtggtgtgatctcggaatttggaaatttgagggctgtatatcacctcatttcgtgtgtccgaatttctacagact

SEQ ID NO: 29 - DNA, 670 bp, Botrytis cinerea
agagcatttgtaggggaaggaggaaaaattgaggaggaggataagatgaattttgataaatttatttcctaacatcaggtcacaatctatgaattacatttgatagtattacgtatgccggtctgtacacaacacaaccatatagtaaggtatcaatcaaatgcgatggatagtcatttcaatttcttagtgaataattacaacgaaccagtaaaatagcaataactctgaaaagcttccggactgccaaaaggtctccaggacgagattattacgaagaacccaagaattcgcctaggaaccaagataaacaaatcatcgacgtgttgcacttccatctatgcgacaattatgccaagcgagccgccagttcttgggggtggagcgctaggaatagggggccggattgccatatccttatctagatctagatggtatcgatatgataaatcaatgcaatggagagttaaaaagttatatgccatatgattgataattattgacaatgcaggctatcgcgggacaatggtaaatggttgtaaaatatggagtctatttccttagctagcgataagatgggtggtttaaacacatcccgccttctctttatcattctccttctcgtattcatatatcataattgcaaagtaaggttgtattttggactgtg

SEQ ID NO: 30 - DNA, 345 bp, Verticillium dahilae
aagctgtcaattgatgcggagggtgagtgaacgtctcgtcggcggggccccttgaggcgagcgcccgttggggggtgttgtggcactaggttctctaggccggcggtgactttcattactatattagaagcaaatacggcgccttcatcacaataataaatatcgatctcgagtcgattccagacccgttataaacctatgtctgtgcaaccagttgggtgctaatttcttgcattatcatcatggatgttgtctatttgagtctcaggtccagctggtgcttataggtcatctccagtatgcgactacctctctccctctttgccattcctaactgattctaac

SEQ ID NO: 31 - DNA, 1000 bp, Verticillium dahilae
cttcatcttccaaccgccattacctcccccatacgcgtcctgccaaagaatcataactggctaaaacataagacgggactggtcatccgctgaaccattccgagctatgtgtcctgattgacccatctcggcttattcgctctcaaatacgactgcaatcgcgtgtggcttggaaaccgtggaataccatcctcatattgtcagcacctgtagcgatacagcacaatgcttgacgattcggaatcattttccgcttctttgcggagcagcggatgtccaattgacgatgacttgactccagaaccaacgtccgaatcacgcgactcaacctccctaccgtatggccttcaggacgacatcggcccccttgctgccaccccgagccagtcgagtaacgtcacaatcaatgcacgggcataccagttggagatgctggcggaaagtaggaagaggaatatcattctagctgtgcgaaccttccctcttgcgccagtcaacctcgattgacacctccatagatggacacaggcagtggcaagacccaagtgtacgttccctgcaagccgaacctgattattgatactgattttcccagtgccgtcctccgaattcgagcagagctagaagaaggggcttcagacaaggtttgacaaactccacttggtagcttcgcaatcacttacagggttttagcttgtatggttcgtggctcacaatgttgagctttgcgctcagcagcattctgtactgcagtctcagattcctgcagttcagaccaagctgcttcttggcagcgataatgttgattcatggtccaaccaagagacttggaacgctgtgcttctcaacgtcaaaattgtggtgtcaacccctcaagttctctgcgatgccttgagccacggctttgtccagatgggttcattatccttgcttgtctttgatgaaggtattcaatcagcgcagtttatcaagtgttcttgccctaacaacggtgtagcgc

SEQ ID NO: 32 - DNA, 25 bp, Verticillium dahilae
taaggatcggaggttcgaatcagtt

SEQ ID NO: 33 - DNA, 26 bp, Verticillium dahilae
gcgaggtgagaggacgaccagccaag

SEQ ID NO: 34 - DNA, 26 bp, Verticillium dahilae
catctgagaggacgtcccgccatggc

SEQ ID NO: 35 - DNA, 26 bp, Verticillium dahilae
gtccgggaaatgaccagcttgagcag

SEQ ID NO: 36 - DNA, 28 bp, Verticillium dahilae
atgtcgatggtcggatgtatccttttct

SEQ ID NO: 37 - DNA, 18 bp, Verticillium dahilae
gattggaacctcagatcc

SEQ ID NO: 38 - DNA, 18 bp, Verticillium dahilae
gcttggaacctctgatcc

SEQ ID NO: 39 - DNA, 18 bp, Verticillium dahilae
gactctaaccttcgatct

SEQ ID NO: 40 - DNA, 19 bp, Verticillium dahilae
tggttggaatctctggtcc

SEQ ID NO: 41 - DNA, 19 bp, Verticillium dahilae
tggttggaatctctggtcc

SEQ ID NO: 42 - DNA, 18 bp, Verticillium dahilae
ctggtcctcctctcacca

SEQ ID NO: 43 - DNA, 18 bp, Verticillium dahilae
ggtggaacttcttctcag

SEQ ID NO: 44 - DNA, 19 bp, Verticillium dahilae
ttcaacctggtgatttctc

SEQ ID NO: 45 - DNA, 19 bp, Verticillium dahilae
ttcaacctggtgatttctc

SEQ ID NO: 46 - DNA, 19 bp, Verticillium dahilae
ttcaacctggtgatttctc

SEQ ID NO: 47 - DNA, 19 bp, Verticillium dahilae
gtcagactggtcatttcca

SEQ ID NO: 48 - DNA, 22 bp, Verticillium dahilae
aaaaagatgcatccgatcttcg

SEQ ID NO: 49 - DNA, 22 bp, Verticillium dahilae
taaaagatatattcgaccatcc

SEQ ID NO: 50 - DNA, 56 bp, Botrytis cinerea
ggggacaagtttgtacaaaaaagcaggcttgcggaagaacttgaaggtttgctaca

SEQ ID NO: 51 - DNA, 25 bp, Botrytis cinerea
gtccagatctggtcaacacaccaag

SEQ ID NO: 52 - DNA, 45 bp, Botrytis cinerea
cttggtgtgttgaccagatctggacggatgccatttgctgcacgc

SEQ ID NO: 53 - DNA, 55 bp, Botrytis cinerea
ggggaccactttgtacaagaaagctgggtactcttgagtactttcgccagctcac

SEQ ID NO: 54 - DNA, 18 bp, Verticillium dahilae
ggatcggaggttcgaatc

SEQ ID NO: 55 - DNA, 18 bp, Verticillium dahilae
ggatcggaggttcgaatc

SEQ ID NO: 56 - DNA, 18 bp, Verticillium dahilae
ggatcggaggttcgaatc

SEQ ID NO: 57 - DNA, 19 bp, Verticillium dahilae
ggatcggaggttcgaatca

SEQ ID NO: 58 - DNA, 19 bp, Verticillium dahilae
ggatcggaggttcgaatca

SEQ ID NO: 59 - DNA, 18 bp, Verticillium dahilae
aggtgagaggacgaccag

SEQ ID NO: 60 - DNA, 18 bp, Verticillium dahilae
ctgagaggacgtcccgcc

SEQ ID NO: 61 - DNA, 19 bp, Verticillium dahilae
gggaaatgaccagcttgag

SEQ ID NO: 62 - DNA, 19 bp, Verticillium dahilae
gggaaatgaccagcttgag

SEQ ID NO: 63 - DNA, 19 bp, Verticillium dahilae
gggaaatgaccagcttgag

SEQ ID NO: 64 - DNA, 19 bp, Verticillium dahilae
gggaaatgaccagcttgag

SEQ ID NO: 65 - DNA, 22 bp, Verticillium dahilae
cgatggtcggatgtatcctttt

SEQ ID NO: 66 - DNA, 22 bp, Verticillium dahilae
cgatggtcggatgtatcctttt